European Patent Application EP 4 674 480 A2, published January 7, 2026. Title: METHODS OF USING ACTIVIN RECEPTOR TYPE II VARIANTS. Applicant: KEROS THERAPEUTICS, INC. Application EP 25196854.1, filed October 1, 2021. The sequence listing filed with the application follows.

SEQUENCE LISTING (385 sequences)

SEQ ID NO: 1 - protein, 109 aa, synthetic construct
  REGION 1..109: note = Synthetic Construct
  VARIANT 14: note = MISC_FEATURE - Xaa is Phe or Tyr
  VARIANT 15: note = MISC_FEATURE - Xaa is Phe or Tyr
  VARIANT 20: note = MISC_FEATURE - Xaa is Glu or Ala
  VARIANT 21: note = MISC_FEATURE - Xaa is Lys or Leu
  VARIANT 22: note = MISC_FEATURE - Xaa is Asp or Glu
  VARIANT 23: note = MISC_FEATURE - Xaa is Arg or Ala
  VARIANT 31: note = MISC_FEATURE - Xaa is Pro or Arg
  VARIANT 33: note = MISC_FEATURE - Xaa is Tyr or Glu
  VARIANT 35: note = MISC_FEATURE - Xaa is Asp or Glu
  VARIANT 36: note = MISC_FEATURE - Xaa is Lys or Gln
  VARIANT 37: note = MISC_FEATURE - Xaa is Asp or Ala
  VARIANT 38: note = MISC_FEATURE - Xaa is Lys or Ala
  VARIANT 39: note = MISC_FEATURE - Xaa is Arg or Ala
  VARIANT 40: note = MISC_FEATURE - Xaa is Arg or Leu
  VARIANT 43: note = MISC_FEATURE - Xaa is Phe or Tyr
  VARIANT 47: note = MISC_FEATURE - Xaa is Lys, Arg, or Ala
  VARIANT 57: note = MISC_FEATURE - Xaa is Lys, Ala, Tyr, Phe, or Ile
  VARIANT 58: note = MISC_FEATURE - Xaa is Gln or Lys
  VARIANT 61: note = MISC_FEATURE - Xaa is Trp or Ala
  VARIANT 62: note = MISC_FEATURE - Xaa is Leu or Ala
  VARIANT 63: note = MISC_FEATURE - Xaa is Asp, Lys, Arg, Ala, Phe, Gly, Met, Asn, or Ile
  VARIANT 65: note = MISC_FEATURE - Xaa is Ile, Phe, or Ala
  VARIANT 76: note = MISC_FEATURE - Xaa is Lys or Thr
  VARIANT 77: note = MISC_FEATURE - Xaa is Lys or Glu
  VARIANT 78: note = MISC_FEATURE - Xaa is Asp or Glu
  VARIANT 79: note = MISC_FEATURE - Xaa is Ser or Asn
  VARIANT 81: note = MISC_FEATURE - Xaa is Glu or Gln
GAILGRSETQECLXXNANWXXXXTNQTGVEXCXGXXXXXXHCXATWXNISGSIEIVXXGCXXXDXNCYDRTDCVEXXXXPXVYFCCCEGNMCNEKFSYFPEMEVTQPTS

SEQ ID NO: 2 - protein, 109 aa, synthetic construct
  REGION 1..109: note = Synthetic Construct
  VARIANT 15: note = MISC_FEATURE - Xaa is Phe or Tyr
  VARIANT 20: note = MISC_FEATURE - Xaa is Glu or Ala
  VARIANT 21: note = MISC_FEATURE - Xaa is Lys or Leu
  VARIANT 22: note = MISC_FEATURE - Xaa is Asp or Glu
  VARIANT 23: note = MISC_FEATURE - Xaa is Arg or Ala
  VARIANT 31: note = MISC_FEATURE - Xaa is Pro or Arg
  VARIANT 33: note = MISC_FEATURE - Xaa is Tyr or Glu
  VARIANT 35: note = MISC_FEATURE - Xaa is Asp or Glu
  VARIANT 37: note = MISC_FEATURE - Xaa is Asp or Ala
  VARIANT 38: note = MISC_FEATURE - Xaa is Lys or Ala
  VARIANT 39: note = MISC_FEATURE - Xaa is Arg or Ala
  VARIANT 40: note = MISC_FEATURE - Xaa is Arg or Leu
  VARIANT 43: note = MISC_FEATURE - Xaa is Phe or Tyr
  VARIANT 47: note = MISC_FEATURE - Xaa is Lys, Arg, or Ala
  VARIANT 57: note = MISC_FEATURE - Xaa is Lys, Ala, Tyr, Phe, or Ile
  VARIANT 58: note = MISC_FEATURE - Xaa is Gln or Lys
  VARIANT 61: note = MISC_FEATURE - Xaa is Trp or Ala
  VARIANT 62: note = MISC_FEATURE - Xaa is Leu or Ala
  VARIANT 63: note = MISC_FEATURE - Xaa is Asp, Lys, Arg, Ala, Phe, Gly, Met, Asn, or Ile
  VARIANT 65: note = MISC_FEATURE - Xaa is Ile, Phe, or Ala
  VARIANT 76: note = MISC_FEATURE - Xaa is Lys or Thr
  VARIANT 77: note = MISC_FEATURE - Xaa is Lys or Glu
  VARIANT 78: note = MISC_FEATURE - Xaa is Asp or Glu
  VARIANT 79: note = MISC_FEATURE - Xaa is Ser or Asn
  VARIANT 81: note = MISC_FEATURE - Xaa is Glu or Gln
GAILGRSETQECLFXNANWXXXXTNQTGVEXCXGXKXXXXHCXATWXNISGSIEIVXXGCXXXDXNCYDRTDCVEXXXXPXVYFCCCEGNMCNEKFSYFPEMEVTQPTS

SEQ ID NO: 3 - protein, 109 aa, synthetic construct
  REGION 1..109: note = Synthetic Construct
  VARIANT 15: note = MISC_FEATURE - Xaa is Phe or Tyr
  VARIANT 21: note = MISC_FEATURE - Xaa is Lys or Leu
  VARIANT 22: note = MISC_FEATURE - Xaa is Asp or Glu
  VARIANT 31: note = MISC_FEATURE - Xaa is Pro or Arg
  VARIANT 33: note = MISC_FEATURE - Xaa is Tyr or Glu
  VARIANT 35: note = MISC_FEATURE - Xaa is Asp or Glu
  VARIANT 40: note = MISC_FEATURE - Xaa is Arg or Leu
  VARIANT 43: note = MISC_FEATURE - Xaa is Phe or Tyr
  VARIANT 47: note = MISC_FEATURE - Xaa is Lys, Arg, or Ala
  VARIANT 58: note = MISC_FEATURE - Xaa is Gln or Lys
  VARIANT 65: note = MISC_FEATURE - Xaa is Ile, Phe, or Ala
  VARIANT 76: note = MISC_FEATURE - Xaa is Lys or Thr
  VARIANT 77: note = MISC_FEATURE - Xaa is Lys or Glu
  VARIANT 78: note = MISC_FEATURE - Xaa is Asp or Glu
  VARIANT 79: note = MISC_FEATURE - Xaa is Ser or Asn
  VARIANT 81: note = MISC_FEATURE - Xaa is Glu or Gln
GAILGRSETQECLFXNANWEXXRTNQTGVEXCXGXKDKRXHCXATWXNISGSIEIVKXGCWLDDXNCYDRTDCVEXXXXPXVYFCCCEGNMCNEKFSYFPEMEVTQPTS

SEQ ID NO: 4 - protein, 109 aa, synthetic construct
  REGION 1..109: note = Synthetic Construct
  VARIANT 15: note = MISC_FEATURE - Xaa is Phe or Tyr
  VARIANT 21: note = MISC_FEATURE - Xaa is Lys or Leu
  VARIANT 31: note = MISC_FEATURE - Xaa is Pro or Arg
  VARIANT 33: note = MISC_FEATURE - Xaa is Tyr or Glu
  VARIANT 35: note = MISC_FEATURE - Xaa is Asp or Glu
  VARIANT 40: note = MISC_FEATURE - Xaa is Arg or Leu
  VARIANT 43: note = MISC_FEATURE - Xaa is Phe or Tyr
  VARIANT 47: note = MISC_FEATURE - Xaa is Lys, Arg, or Ala
  VARIANT 58: note = MISC_FEATURE - Xaa is Gln or Lys
  VARIANT 65: note = MISC_FEATURE - Xaa is Ile, Phe, or Ala
  VARIANT 76: note = MISC_FEATURE - Xaa is Lys or Thr
  VARIANT 78: note = MISC_FEATURE - Xaa is Asp or Glu
  VARIANT 79: note = MISC_FEATURE - Xaa is Ser or Asn
  VARIANT 81: note = MISC_FEATURE - Xaa is Glu or Gln
GAILGRSETQECLFXNANWEXDRTNQTGVEXCXGXKDKRXHCXATWXNISGSIEIVKXGCWLDDXNCYDRTDCVEXKXXPXVYFCCCEGNMCNEKFSYFPEMEVTQPTS

SEQ ID NO: 5 - protein, 109 aa, synthetic construct
  REGION 1..109: note = Synthetic Construct
  VARIANT 15: note = MISC_FEATURE - Xaa is Phe or Tyr
  VARIANT 21: note = MISC_FEATURE - Xaa is Lys or Leu
  VARIANT 33: note = MISC_FEATURE - Xaa is Tyr or Glu
  VARIANT 35: note = MISC_FEATURE - Xaa is Asp or Glu
  VARIANT 40: note = MISC_FEATURE - Xaa is Arg or Leu
  VARIANT 58: note = MISC_FEATURE - Xaa is Gln or Lys
  VARIANT 76: note = MISC_FEATURE - Xaa is Lys or Thr
  VARIANT 78: note = MISC_FEATURE - Xaa is Asp or Glu
  VARIANT 79: note = MISC_FEATURE - Xaa is Ser or Asn
  VARIANT 81: note = MISC_FEATURE - Xaa is Glu or Gln
GAILGRSETQECLFXNANWEXDRTNQTGVEPCXGXKDKRXHCFATWKNISGSIEIVKXGCWLDDINCYDRTDCVEXKXXPXVYFCCCEGNMCNEKFSYFPEMEVTQPTS

SEQ ID NO: 6 - protein, 109 aa, synthetic construct
  REGION 1..109: note = Synthetic Construct
GAILGRSETQECLFYNANWELDRTNQTGVEPCEGEKDKRLHCFATWKNISGSIEIVKKGCWLDDINCYDRTDCVETKENPQVYFCCCEGNMCNEKFSYFPEMEVTQPTS

SEQ ID NO: 7 - protein, 109 aa, synthetic construct
  REGION 1..109: note = Synthetic Construct
GAILGRSETQECLFYNANWELERTNQTGVEPCEGEKDKRLHCFATWKNISGSIEIVKKGCWLDDINCYDRTDCVETKENPQVYFCCCEGNMCNEKFSYFPEMEVTQPTS

SEQ ID NO: 8 - protein, 109 aa, synthetic construct
  REGION 1..109: note = Synthetic Construct
GAILGRSETQECLFYNANWELDRTNQTGVERCEGEKDKRLHCFATWKNISGSIEIVKKGCWLDDINCYDRTDCVETKENPQVYFCCCEGNMCNEKFSYFPEMEVTQPTS

SEQ ID NO: 9 - protein, 109 aa, synthetic construct
  REGION 1..109: note = Synthetic Construct
GAILGRSETQECLFYNANWELDRTNQTGVEPCEGEKDKRLHCYATWKNISGSIEIVKKGCWLDDINCYDRTDCVETKENPQVYFCCCEGNMCNEKFSYFPEMEVTQPTS

SEQ ID NO: 10 - protein, 109 aa, synthetic construct
  REGION 1..109: note = Synthetic Construct
GAILGRSETQECLFYNANWELDRTNQTGVEPCEGEKDKRLHCFATWRNISGSIEIVKKGCWLDDINCYDRTDCVETKENPQVYFCCCEGNMCNEKFSYFPEMEVTQPTS

SEQ ID NO: 11 - protein, 109 aa, synthetic construct
  REGION 1..109: note = Synthetic Construct
GAILGRSETQECLFYNANWELDRTNQTGVEPCEGEKDKRLHCFATWKNISGSIEIVKKGCWLDDFNCYDRTDCVETKENPQVYFCCCEGNMCNEKFSYFPEMEVTQPTS

SEQ ID NO: 12 - protein, 109 aa, synthetic construct
  REGION 1..109: note = Synthetic Construct
GAILGRSETQECLFYNANWELDRTNQTGVEPCEGEKDKRLHCFATWKNISGSIEIVKKGCWLDDINCYDRTDCVETEENPQVYFCCCEGNMCNEKFSYFPEMEVTQPTS

SEQ ID NO: 13 - protein, 109 aa, synthetic construct
  REGION 1..109: note = Synthetic Construct
GAILGRSETQECLFYNANWELERTNQTGVERCEGEKDKRLHCFATWKNISGSIEIVKKGCWLDDINCYDRTDCVETKENPQVYFCCCEGNMCNEKFSYFPEMEVTQPTS

SEQ ID NO: 14 - protein, 109 aa, synthetic construct
  REGION 1..109: note = Synthetic Construct
GAILGRSETQECLFYNANWELERTNQTGVEPCEGEKDKRLHCYATWKNISGSIEIVKKGCWLDDINCYDRTDCVETKENPQVYFCCCEGNMCNEKFSYFPEMEVTQPTS

SEQ ID NO: 15 - protein, 109 aa, synthetic construct
  REGION 1..109: note = Synthetic Construct
GAILGRSETQECLFYNANWELERTNQTGVEPCEGEKDKRLHCFATWRNISGSIEIVKKGCWLDDINCYDRTDCVETKENPQVYFCCCEGNMCNEKFSYFPEMEVTQPTS

SEQ ID NO: 16 - protein, 109 aa, synthetic construct
  REGION 1..109: note = Synthetic Construct
GAILGRSETQECLFYNANWELERTNQTGVEPCEGEKDKRLHCFATWKNISGSIEIVKKGCWLDDFNCYDRTDCVETKENPQVYFCCCEGNMCNEKFSYFPEMEVTQPTS

SEQ ID NO: 17 - protein, 109 aa, synthetic construct
  REGION 1..109: note = Synthetic Construct
GAILGRSETQECLFYNANWELERTNQTGVEPCEGEKDKRLHCFATWKNISGSIEIVKKGCWLDDINCYDRTDCVETEENPQVYFCCCEGNMCNEKFSYFPEMEVTQPTS

SEQ ID NO: 18 - protein, 109 aa, synthetic construct
  REGION 1..109: note = Synthetic Construct
GAILGRSETQECLFYNANWELDRTNQTGVERCEGEKDKRLHCYATWKNISGSIEIVKKGCWLDDINCYDRTDCVETKENPQVYFCCCEGNMCNEKFSYFPEMEVTQPTS

SEQ ID NO: 19 - protein, 109 aa, synthetic construct
  REGION 1..109: note = Synthetic Construct
GAILGRSETQECLFYNANWELDRTNQTGVERCEGEKDKRLHCFATWRNISGSIEIVKKGCWLDDINCYDRTDCVETKENPQVYFCCCEGNMCNEKFSYFPEMEVTQPTS

SEQ ID NO: 20 - protein, 109 aa, synthetic construct
  REGION 1..109: note = Synthetic Construct
GAILGRSETQECLFYNANWELDRTNQTGVERCEGEKDKRLHCFATWKNISGSIEIVKKGCWLDDFNCYDRTDCVETKENPQVYFCCCEGNMCNEKFSYFPEMEVTQPTS

SEQ ID NO: 21 - protein, 109 aa, synthetic construct
  REGION 1..109: note = Synthetic Construct
GAILGRSETQECLFYNANWELDRTNQTGVERCEGEKDKRLHCFATWKNISGSIEIVKKGCWLDDINCYDRTDCVETEENPQVYFCCCEGNMCNEKFSYFPEMEVTQPTS

SEQ ID NO: 22 - protein, 109 aa, synthetic construct
  REGION 1..109: note = Synthetic Construct
GAILGRSETQECLFYNANWELDRTNQTGVEPCEGEKDKRLHCYATWRNISGSIEIVKKGCWLDDINCYDRTDCVETKENPQVYFCCCEGNMCNEKFSYFPEMEVTQPTS

SEQ ID NO: 23 - protein, 109 aa, synthetic construct
  REGION 1..109: note = Synthetic Construct
GAILGRSETQECLFYNANWELDRTNQTGVEPCEGEKDKRLHCYATWKNISGSIEIVKKGCWLDDFNCYDRTDCVETKENPQVYFCCCEGNMCNEKFSYFPEMEVTQPTS

SEQ ID NO: 24 - protein, 109 aa, synthetic construct
  REGION 1..109: note = Synthetic Construct
GAILGRSETQECLFYNANWELDRTNQTGVEPCEGEKDKRLHCYATWKNISGSIEIVKKGCWLDDINCYDRTDCVETEENPQVYFCCCEGNMCNEKFSYFPEMEVTQPTS

SEQ ID NO: 25 - protein, 109 aa, synthetic construct
  REGION 1..109: note = Synthetic Construct
GAILGRSETQECLFYNANWELDRTNQTGVEPCEGEKDKRLHCFATWRNISGSIEIVKKGCWLDDFNCYDRTDCVETKENPQVYFCCCEGNMCNEKFSYFPEMEVTQPTS

SEQ ID NO: 26 - protein, 109 aa, synthetic construct
  REGION 1..109: note = Synthetic Construct
GAILGRSETQECLFYNANWELDRTNQTGVEPCEGEKDKRLHCFATWRNISGSIEIVKKGCWLDDINCYDRTDCVETEENPQVYFCCCEGNMCNEKFSYFPEMEVTQPTS

SEQ ID NO: 27 - protein, 109 aa, synthetic construct
  REGION 1..109: note = Synthetic Construct
GAILGRSETQECLFYNANWELDRTNQTGVEPCEGEKDKRLHCFATWKNISGSIEIVKKGCWLDDFNCYDRTDCVETEENPQVYFCCCEGNMCNEKFSYFPEMEVTQPTS

SEQ ID NO: 28 - protein, 109 aa, synthetic construct
  REGION 1..109: note = Synthetic Construct
GAILGRSETQECLFYNANWELERTNQTGVERCEGEKDKRLHCYATWKNISGSIEIVKKGCWLDDINCYDRTDCVETKENPQVYFCCCEGNMCNEKFSYFPEMEVTQPTS

SEQ ID NO: 29 - protein, 109 aa, synthetic construct
  REGION 1..109: note = Synthetic Construct
GAILGRSETQECLFYNANWELERTNQTGVERCEGEKDKRLHCFATWRNISGSIEIVKKGCWLDDINCYDRTDCVETKENPQVYFCCCEGNMCNEKFSYFPEMEVTQPTS

SEQ ID NO: 30 - protein, 109 aa, synthetic construct
  REGION 1..109: note = Synthetic Construct
GAILGRSETQECLFYNANWELERTNQTGVERCEGEKDKRLHCFATWKNISGSIEIVKKGCWLDDFNCYDRTDCVETKENPQVYFCCCEGNMCNEKFSYFPEMEVTQPTS

SEQ ID NO: 31 - protein, 109 aa, synthetic construct
  REGION 1..109: note = Synthetic Construct
GAILGRSETQECLFYNANWELERTNQTGVERCEGEKDKRLHCFATWKNISGSIEIVKKGCWLDDINCYDRTDCVETEENPQVYFCCCEGNMCNEKFSYFPEMEVTQPTS

SEQ ID NO: 32 - protein, 109 aa, synthetic construct
  REGION 1..109: note = Synthetic Construct
GAILGRSETQECLFYNANWELERTNQTGVEPCEGEKDKRLHCYATWRNISGSIEIVKKGCWLDDINCYDRTDCVETKENPQVYFCCCEGNMCNEKFSYFPEMEVTQPTS

SEQ ID NO: 33 - protein, 109 aa, synthetic construct
  REGION 1..109: note = Synthetic Construct
GAILGRSETQECLFYNANWELERTNQTGVEPCEGEKDKRLHCYATWKNISGSIEIVKKGCWLDDFNCYDRTDCVETKENPQVYFCCCEGNMCNEKFSYFPEMEVTQPTS

SEQ ID NO: 34 - protein, 109 aa, synthetic construct
  REGION 1..109: note = Synthetic Construct
GAILGRSETQECLFYNANWELERTNQTGVEPCEGEKDKRLHCYATWKNISGSIEIVKKGCWLDDINCYDRTDCVETEENPQVYFCCCEGNMCNEKFSYFPEMEVTQPTS

SEQ ID NO: 35 - protein, 109 aa, synthetic construct
  REGION 1..109: note = Synthetic Construct
GAILGRSETQECLFYNANWELERTNQTGVEPCEGEKDKRLHCFATWRNISGSIEIVKKGCWLDDFNCYDRTDCVETKENPQVYFCCCEGNMCNEKFSYFPEMEVTQPTS

SEQ ID NO: 36 - protein, 109 aa, synthetic construct
  REGION 1..109: note = Synthetic Construct
GAILGRSETQECLFYNANWELERTNQTGVEPCEGEKDKRLHCFATWRNISGSIEIVKKGCWLDDINCYDRTDCVETEENPQVYFCCCEGNMCNEKFSYFPEMEVTQPTS

SEQ ID NO: 37 - protein, 109 aa, synthetic construct
  REGION 1..109: note = Synthetic Construct
GAILGRSETQECLFYNANWELERTNQTGVEPCEGEKDKRLHCFATWKNISGSIEIVKKGCWLDDFNCYDRTDCVETEENPQVYFCCCEGNMCNEKFSYFPEMEVTQPTS

SEQ ID NO: 38 - protein, 109 aa, synthetic construct
  REGION 1..109: note = Synthetic Construct
GAILGRSETQECLFYNANWELDRTNQTGVERCEGEKDKRLHCYATWRNISGSIEIVKKGCWLDDINCYDRTDCVETKENPQVYFCCCEGNMCNEKFSYFPEMEVTQPTS

SEQ ID NO: 39 - protein, 109 aa, synthetic construct
  REGION 1..109: note = Synthetic Construct
GAILGRSETQECLFYNANWELDRTNQTGVERCEGEKDKRLHCYATWKNISGSIEIVKKGCWLDDFNCYDRTDCVETKENPQVYFCCCEGNMCNEKFSYFPEMEVTQPTS

SEQ ID NO: 40 - protein, 109 aa, synthetic construct
  REGION 1..109: note = Synthetic Construct
GAILGRSETQECLFYNANWELDRTNQTGVERCEGEKDKRLHCYATWKNISGSIEIVKKGCWLDDINCYDRTDCVETEENPQVYFCCCEGNMCNEKFSYFPEMEVTQPTS

SEQ ID NO: 41 - protein, 109 aa, synthetic construct
  REGION 1..109: note = Synthetic Construct
GAILGRSETQECLFYNANWELDRTNQTGVERCEGEKDKRLHCFATWRNISGSIEIVKKGCWLDDFNCYDRTDCVETKENPQVYFCCCEGNMCNEKFSYFPEMEVTQPTS

SEQ ID NO: 42 - protein, 109 aa, synthetic construct
  REGION 1..109: note = Synthetic Construct
GAILGRSETQECLFYNANWELDRTNQTGVERCEGEKDKRLHCFATWRNISGSIEIVKKGCWLDDINCYDRTDCVETEENPQVYFCCCEGNMCNEKFSYFPEMEVTQPTS

SEQ ID NO: 43 - protein, 109 aa, synthetic construct
  REGION 1..109: note = Synthetic Construct
GAILGRSETQECLFYNANWELDRTNQTGVERCEGEKDKRLHCFATWKNISGSIEIVKKGCWLDDFNCYDRTDCVETEENPQVYFCCCEGNMCNEKFSYFPEMEVTQPTS

SEQ ID NO: 44 - protein, 109 aa, synthetic construct
  REGION 1..109: note = Synthetic Construct
GAILGRSETQECLFYNANWELDRTNQTGVEPCEGEKDKRLHCYATWRNISGSIEIVKKGCWLDDFNCYDRTDCVETKENPQVYFCCCEGNMCNEKFSYFPEMEVTQPTS

SEQ ID NO: 45 - protein, 109 aa, synthetic construct
  REGION 1..109: note = Synthetic Construct
GAILGRSETQECLFYNANWELDRTNQTGVEPCEGEKDKRLHCYATWRNISGSIEIVKKGCWLDDINCYDRTDCVETEENPQVYFCCCEGNMCNEKFSYFPEMEVTQPTS

SEQ ID NO: 46 - protein, 109 aa, synthetic construct
  REGION 1..109: note = Synthetic Construct
GAILGRSETQECLFYNANWELDRTNQTGVEPCEGEKDKRLHCYATWKNISGSIEIVKKGCWLDDFNCYDRTDCVETEENPQVYFCCCEGNMCNEKFSYFPEMEVTQPTS

SEQ ID NO: 47 - protein, 109 aa, synthetic construct
  REGION 1..109: note = Synthetic Construct
GAILGRSETQECLFYNANWELDRTNQTGVEPCEGEKDKRLHCFATWRNISGSIEIVKKGCWLDDFNCYDRTDCVETEENPQVYFCCCEGNMCNEKFSYFPEMEVTQPTS

SEQ ID NO: 48 - protein, 109 aa, synthetic construct
  REGION 1..109: note = Synthetic Construct
GAILGRSETQECLFYNANWELERTNQTGVERCEGEKDKRLHCYATWRNISGSIEIVKKGCWLDDINCYDRTDCVETKENPQVYFCCCEGNMCNEKFSYFPEMEVTQPTS

SEQ ID NO: 49 - protein, 109 aa, synthetic construct
  REGION 1..109: note = Synthetic Construct
GAILGRSETQECLFYNANWELERTNQTGVERCEGEKDKRLHCYATWKNISGSIEIVKKGCWLDDFNCYDRTDCVETKENPQVYFCCCEGNMCNEKFSYFPEMEVTQPTS

SEQ ID NO: 50 - protein, 109 aa, synthetic construct
  REGION 1..109: note = Synthetic Construct
GAILGRSETQECLFYNANWELERTNQTGVERCEGEKDKRLHCYATWKNISGSIEIVKKGCWLDDINCYDRTDCVETEENPQVYFCCCEGNMCNEKFSYFPEMEVTQPTS

SEQ ID NO: 51 - protein, 109 aa, synthetic construct
  REGION 1..109: note = Synthetic Construct
GAILGRSETQECLFYNANWELERTNQTGVERCEGEKDKRLHCFATWRNISGSIEIVKKGCWLDDFNCYDRTDCVETKENPQVYFCCCEGNMCNEKFSYFPEMEVTQPTS

SEQ ID NO: 52 - protein, 109 aa, synthetic construct
  REGION 1..109: note = Synthetic Construct
GAILGRSETQECLFYNANWELERTNQTGVERCEGEKDKRLHCFATWRNISGSIEIVKKGCWLDDINCYDRTDCVETEENPQVYFCCCEGNMCNEKFSYFPEMEVTQPTS

SEQ ID NO: 53 - protein, 109 aa, synthetic construct
  REGION 1..109: note = Synthetic Construct
GAILGRSETQECLFYNANWELERTNQTGVERCEGEKDKRLHCFATWKNISGSIEIVKKGCWLDDFNCYDRTDCVETEENPQVYFCCCEGNMCNEKFSYFPEMEVTQPTS

SEQ ID NO: 54 - protein, 109 aa, synthetic construct
  REGION 1..109: note = Synthetic Construct
GAILGRSETQECLFYNANWELERTNQTGVEPCEGEKDKRLHCYATWRNISGSIEIVKKGCWLDDFNCYDRTDCVETKENPQVYFCCCEGNMCNEKFSYFPEMEVTQPTS

SEQ ID NO: 55 - protein, 109 aa, synthetic construct
  REGION 1..109: note = Synthetic Construct
GAILGRSETQECLFYNANWELERTNQTGVEPCEGEKDKRLHCYATWRNISGSIEIVKKGCWLDDINCYDRTDCVETEENPQVYFCCCEGNMCNEKFSYFPEMEVTQPTS

SEQ ID NO: 56 - protein, 109 aa, synthetic construct
  REGION 1..109: note = Synthetic Construct
GAILGRSETQECLFYNANWELERTNQTGVEPCEGEKDKRLHCYATWKNISGSIEIVKKGCWLDDFNCYDRTDCVETEENPQVYFCCCEGNMCNEKFSYFPEMEVTQPTS

SEQ ID NO: 57 - protein, 109 aa, synthetic construct
  REGION 1..109: note = Synthetic Construct
GAILGRSETQECLFYNANWELERTNQTGVEPCEGEKDKRLHCFATWRNISGSIEIVKKGCWLDDFNCYDRTDCVETEENPQVYFCCCEGNMCNEKFSYFPEMEVTQPTS

SEQ ID NO: 58 - protein, 109 aa, synthetic construct
  REGION 1..109: note = Synthetic Construct
GAILGRSETQECLFYNANWELDRTNQTGVERCEGEKDKRLHCYATWRNISGSIEIVKKGCWLDDFNCYDRTDCVETKENPQVYFCCCEGNMCNEKFSYFPEMEVTQPTS

SEQ ID NO: 59 - protein, 109 aa, synthetic construct
  REGION 1..109: note = Synthetic Construct
GAILGRSETQECLFYNANWELDRTNQTGVERCEGEKDKRLHCYATWRNISGSIEIVKKGCWLDDINCYDRTDCVETEENPQVYFCCCEGNMCNEKFSYFPEMEVTQPTS

SEQ ID NO: 60 - protein, 109 aa, synthetic construct
  REGION 1..109: note = Synthetic Construct
GAILGRSETQECLFYNANWELDRTNQTGVERCEGEKDKRLHCYATWKNISGSIEIVKKGCWLDDFNCYDRTDCVETEENPQVYFCCCEGNMCNEKFSYFPEMEVTQPTS

SEQ ID NO: 61 - protein, 109 aa, synthetic construct
  REGION 1..109: note = Synthetic Construct
GAILGRSETQECLFYNANWELDRTNQTGVERCEGEKDKRLHCFATWRNISGSIEIVKKGCWLDDFNCYDRTDCVETEENPQVYFCCCEGNMCNEKFSYFPEMEVTQPTS

SEQ ID NO: 62 - protein, 109 aa, synthetic construct
  REGION 1..109: note = Synthetic Construct
GAILGRSETQECLFYNANWELDRTNQTGVEPCEGEKDKRLHCYATWRNISGSIEIVKKGCWLDDFNCYDRTDCVETEENPQVYFCCCEGNMCNEKFSYFPEMEVTQPTS

SEQ ID NO: 63 - protein, 109 aa, synthetic construct
  REGION 1..109: note = Synthetic Construct
GAILGRSETQECLFYNANWELERTNQTGVERCEGEKDKRLHCYATWRNISGSIEIVKKGCWLDDFNCYDRTDCVETKENPQVYFCCCEGNMCNEKFSYFPEMEVTQPTS

SEQ ID NO: 64 - protein, 109 aa, synthetic construct
  REGION 1..109: note = Synthetic Construct
GAILGRSETQECLFYNANWELERTNQTGVERCEGEKDKRLHCYATWRNISGSIEIVKKGCWLDDINCYDRTDCVETEENPQVYFCCCEGNMCNEKFSYFPEMEVTQPTS

SEQ ID NO: 65 - protein, 109 aa, synthetic construct
  REGION 1..109: note = Synthetic Construct
GAILGRSETQECLFYNANWELERTNQTGVERCEGEKDKRLHCYATWKNISGSIEIVKKGCWLDDFNCYDRTDCVETEENPQVYFCCCEGNMCNEKFSYFPEMEVTQPTS

SEQ ID NO: 66 - protein, 109 aa, synthetic construct
  REGION 1..109: note = Synthetic Construct
GAILGRSETQECLFYNANWELERTNQTGVERCEGEKDKRLHCFATWRNISGSIEIVKKGCWLDDFNCYDRTDCVETEENPQVYFCCCEGNMCNEKFSYFPEMEVTQPTS

SEQ ID NO: 67 - protein, 109 aa, synthetic construct
  REGION 1..109: note = Synthetic Construct
GAILGRSETQECLFYNANWELDRTNQTGVERCEGEKDKRLHCYATWRNISGSIEIVKKGCWLDDFNCYDRTDCVETEENPQVYFCCCEGNMCNEKFSYFPEMEVTQPTS

SEQ ID NO: 68 - protein, 109 aa, synthetic construct
  REGION 1..109: note = Synthetic Construct
GAILGRSETQECLFYNANWELERTNQTGVEPCEGEKDKRLHCYATWRNISGSIEIVKKGCWLDDFNCYDRTDCVETEENPQVYFCCCEGNMCNEKFSYFPEMEVTQPTS

SEQ ID NO: 69 - protein, 109 aa, synthetic construct
  REGION 1..109: note = Synthetic Construct
GAILGRSETQECLFYNANWELERTNQTGVERCEGEKDKRLHCYATWRNISGSIEIVKKGCWLDDFNCYDRTDCVETEENPQVYFCCCEGNMCNEKFSYFPEMEVTQPTS

SEQ ID NO: 70 - protein, 109 aa, synthetic construct
  REGION 1..109: note = Synthetic Construct
GAILGRSETQECLYYNANWELERTNQTGVERCEGEQDKRLHCYATWRNISGSIEIVKKGCWLDDFNCYDRTDCVETEENPQVYFCCCEGNMCNEKFSYFPEMEVTQPTS

SEQ ID NO: 71 - protein, 111 aa, synthetic construct
  REGION 1..111: note = Synthetic Construct
GAILGRSETQECLFYNANWELERTNQTGVERCEGEKDKRLHCYATWRNISGSIEIVKKGCWLDDFNCYDRTDCVETEENPQVYFCCCEGNMCNEKFSYFPEMEVTQPTSNP

SEQ ID NO: 72 - protein, 115 aa, synthetic construct
  REGION 1..115: note = Synthetic Construct
GAILGRSETQECLFYNANWELERTNQTGVERCEGEKDKRLHCYATWRNISGSIEIVKKGCWLDDFNCYDRTDCVETEENPQVYFCCCEGNMCNEKFSYFPEMEVTQPTSNPVTPK

SEQ ID NO: 73 - protein, 109 aa, Homo sapiens
GAILGRSETQECLFFNANWEKDRTNQTGVEPCYGDKDKRRHCFATWKNISGSIEIVKQGCWLDDINCYDRTDCVEKKDSPEVYFCCCEGNMCNEKFSYFPEMEVTQPTS

SEQ ID NO: 74 - protein, 115 aa, Homo sapiens
GRGEAETRECIYYNANWELERTNQSGLERCEGEQDKRLHCYASWRNSSGTIELVKKGCWLDDFNCYDRQECVATEENPQVYFCCCEGNFCNERFTHLPEAGGPEVTYEPPPTAPT

SEQ ID NO: 75 - protein, 513 aa, Homo sapiens
MGAAAKLAFAVFLISCSSGAILGRSETQECLFFNANWEKDRTNQTGVEPCYGDKDKRRHCFATWKNISGSIEIVKQGCWLDDINCYDRTDCVEKKDSPEVYFCCCEGNMCNEKFSYFPEMEVTQPTSNPVTPKPPYYNILLYSLVPLMLIAGIVICAFWVYRHHKMAYPPVLVPTQDPGPPPPSPLLGLKPLQLLEVKARGRFGCVWKAQLLNEYVAVKIFPIQDKQSWQNEYEVYSLPGMKHENILQFIGAEKRGTSVDVDLWLITAFHEKGSLSDFLKANVVSWNELCHIAETMARGLAYLHEDIPGLKDGHKPAISHRDIKSKNVLLKNNLTACIADFGLALKFEAGKSAGDTHGQVGTRRYMAPEVLEGAINFQRDAFLRIDMYAMGLVLWELASRCTAADGPVDEYMLPFEEEIGQHPSLEDMQEVVVHKKKRPVLRDYWQKHAGMAMLCETIEECWDHDAEARLSAGCVGERITQMQRLTNIITTEDIVTVVTMVTNVDFPPKESSL

SEQ ID NO: 76 - protein, 109 aa, synthetic construct
  REGION 1..109: note = Synthetic Construct
GAILGRSETQECLFFNANWEKDRTNQTGVEPCYGDKDKRRHCFATWANISGSIEIVKQGCWLDDINCYDRTDCVEKKDSPEVYFCCCEGNMCNEKFSYFPEMEVTQPTS

SEQ ID NO: 77 - protein, 109 aa, synthetic construct
  REGION 1..109: note = Synthetic Construct
GAILGRSETQECLFFNANWAKDRTNQTGVEPCYGDKDKRRHCFATWKNISGSIEIVKQGCWLDDINCYDRTDCVEKKDSPEVYFCCCEGNMCNEKFSYFPEMEVTQPTS

SEQ ID NO: 78 - protein, 109 aa, synthetic construct
  REGION 1..109: note = Synthetic Construct
GAILGRSETQECLFFNANWEKDATNQTGVEPCYGDKDKRRHCFATWKNISGSIEIVKQGCWLDDINCYDRTDCVEKKDSPEVYFCCCEGNMCNEKFSYFPEMEVTQPTS

SEQ ID NO: 79 - protein, 109 aa, synthetic construct
  REGION 1..109: note = Synthetic Construct
GAILGRSETQECLFFNANWEKDRTNQTGVEPCYGDKAKRRHCFATWKNISGSIEIVKQGCWLDDINCYDRTDCVEKKDSPEVYFCCCEGNMCNEKFSYFPEMEVTQPTS

SEQ ID NO: 80 - protein, 109 aa, synthetic construct
  REGION 1..109: note = Synthetic Construct
GAILGRSETQECLFFNANWEKDRTNQTGVEPCYGDKDARRHCFATWKNISGSIEIVKQGCWLDDINCYDRTDCVEKKDSPEVYFCCCEGNMCNEKFSYFPEMEVTQPTS

SEQ ID NO: 81 - protein, 109 aa, synthetic construct
  REGION 1..109: note = Synthetic Construct
GAILGRSETQECLFFNANWEKDRTNQTGVEPCYGDKDKARHCFATWKNISGSIEIVKQGCWLDDINCYDRTDCVEKKDSPEVYFCCCEGNMCNEKFSYFPEMEVTQPTS

SEQ ID NO: 82 - protein, 109 aa, synthetic construct
  REGION 1..109: note = Synthetic Construct
GAILGRSETQECLFFNANWEKDRTNQTGVEPCYGDKDKRRHCFATWKNISGSIEIVAQGCWLDDINCYDRTDCVEKKDSPEVYFCCCEGNMCNEKFSYFPEMEVTQPTS

SEQ ID NO: 83 - protein, 109 aa, synthetic construct
  REGION 1..109: note = Synthetic Construct
GAILGRSETQECLFFNANWEKDRTNQTGVEPCYGDKDKRRHCFATWKNISGSIEIVYQGCWLDDINCYDRTDCVEKKDSPEVYFCCCEGNMCNEKFSYFPEMEVTQPTS

SEQ ID NO: 84 - protein, 109 aa, synthetic construct
  REGION 1..109: note = Synthetic Construct
GAILGRSETQECLFFNANWEKDRTNQTGVEPCYGDKDKRRHCFATWKNISGSIEIVFQGCWLDDINCYDRTDCVEKKDSPEVYFCCCEGNMCNEKFSYFPEMEVTQPTS

SEQ ID NO: 85 - protein, 109 aa, synthetic construct
  REGION 1..109: note = Synthetic Construct
GAILGRSETQECLFFNANWEKDRTNQTGVEPCYGDKDKRRHCFATWKNISGSIEIVIQGCWLDDINCYDRTDCVEKKDSPEVYFCCCEGNMCNEKFSYFPEMEVTQPTS

SEQ ID NO: 86 - protein, 109 aa, synthetic construct
  REGION 1..109: note = Synthetic Construct
GAILGRSETQECLFFNANWEKDRTNQTGVEPCYGDKDKRRHCFATWKNISGSIEIVKQGCALDDINCYDRTDCVEKKDSPEVYFCCCEGNMCNEKFSYFPEMEVTQPTS

SEQ ID NO: 87 - protein, 109 aa, synthetic construct
  REGION 1..109: note = Synthetic Construct
GAILGRSETQECLFFNANWEKDRTNQTGVEPCYGDKDKRRHCFATWKNISGSIEIVKQGCWADDINCYDRTDCVEKKDSPEVYFCCCEGNMCNEKFSYFPEMEVTQPTS

SEQ ID NO: 88 - protein, 109 aa, synthetic construct
  REGION 1..109: note = Synthetic Construct
GAILGRSETQECLFFNANWEKDRTNQTGVEPCYGDKDKRRHCFATWKNISGSIEIVKQGCWLKDINCYDRTDCVEKKDSPEVYFCCCEGNMCNEKFSYFPEMEVTQPTS

SEQ ID NO: 89 - protein, 109 aa, synthetic construct
  REGION 1..109: note = Synthetic Construct
GAILGRSETQECLFFNANWEKDRTNQTGVEPCYGDKDKRRHCFATWKNISGSIEIVKQGCWLRDINCYDRTDCVEKKDSPEVYFCCCEGNMCNEKFSYFPEMEVTQPTS

SEQ ID NO: 90 - protein, 109 aa, synthetic construct
  REGION 1..109: note = Synthetic Construct
GAILGRSETQECLFFNANWEKDRTNQTGVEPCYGDKDKRRHCFATWKNISGSIEIVKQGCWLADINCYDRTDCVEKKDSPEVYFCCCEGNMCNEKFSYFPEMEVTQPTS

SEQ ID NO: 91 - protein, 109 aa, synthetic construct
  REGION 1..109: note = Synthetic Construct
GAILGRSETQECLFFNANWEKDRTNQTGVEPCYGDKDKRRHCFATWKNISGSIEIVKQGCWLFDINCYDRTDCVEKKDSPEVYFCCCEGNMCNEKFSYFPEMEVTQPTS

SEQ ID NO: 92 - protein, 109 aa, synthetic construct
  REGION 1..109: note = Synthetic Construct
GAILGRSETQECLFFNANWEKDRTNQTGVEPCYGDKDKRRHCFATWKNISGSIEIVKQGCWLGDINCYDRTDCVEKKDSPEVYFCCCEGNMCNEKFSYFPEMEVTQPTS

SEQ ID NO: 93 - protein, 109 aa, synthetic construct
  REGION 1..109: note = Synthetic Construct
GAILGRSETQECLFFNANWEKDRTNQTGVEPCYGDKDKRRHCFATWKNISGSIEIVKQGCWLMDINCYDRTDCVEKKDSPEVYFCCCEGNMCNEKFSYFPEMEVTQPTS

SEQ ID NO: 94 - protein, 109 aa, synthetic construct
  REGION 1..109: note = Synthetic Construct
GAILGRSETQECLFFNANWEKDRTNQTGVEPCYGDKDKRRHCFATWKNISGSIEIVKQGCWLNDINCYDRTDCVEKKDSPEVYFCCCEGNMCNEKFSYFPEMEVTQPTS

SEQ ID NO: 95 - protein, 109 aa, synthetic construct
  REGION 1..109: note = Synthetic Construct
GAILGRSETQECLFFNANWEKDRTNQTGVEPCYGDKDKRRHCFATWKNISGSIEIVKQGCWLIDINCYDRTDCVEKKDSPEVYFCCCEGNMCNEKFSYFPEMEVTQPTS

SEQ ID NO: 96 - protein, 109 aa, synthetic construct
  REGION 1..109: note = Synthetic Construct
GAILGRSETQECLFFNANWEKDRTNQTGVEPCYGDKDKRRHCFATWKNISGSIEIVKQGCWLDDANCYDRTDCVEKKDSPEVYFCCCEGNMCNEKFSYFPEMEVTQPTS

SEQ ID NO: 97 - protein, 225 aa, Homo sapiens
THTCPPCPAPELLGGPSVFLFPPKPKDTLMISRTPEVTCVVVDVSHEDPEVKFNWYVDGVEVHNAKTKPREEQYNSTYRVVSVLTVLHQDWLNGKEYKCKVSNKALPVPIEKTISKAKGQPREPQVYTLPPSREEMTKNQVSLTCLVKGFYPSDIAVEWESNGQPENNYKTTPPVLDSDGPFFLYSKLTVDKSRWQQGNVFSCSVMHEALHNHYTQKSLSLSPGK

SEQ ID NO: 98 - protein, 4 aa, synthetic construct
  REGION 1..4: note = Synthetic Construct
GGGA

SEQ ID NO: 99 - protein, 4 aa, synthetic construct
  REGION 1..4: note = Synthetic Construct
GGGS

SEQ ID NO: 100 - protein, 4 aa, synthetic construct
  REGION 1..4: note = Synthetic Construct
GGGG

SEQ ID NO: 101 - protein, 5 aa, synthetic construct
  REGION 1..5: note = Synthetic Construct
GGGGA

SEQ ID NO: 102 - protein, 5 aa, synthetic construct
  REGION 1..5: note = Synthetic Construct
GGGGS

SEQ ID NO: 103 - protein, 5 aa, synthetic construct
  REGION 1..5: note = Synthetic Construct
GGGGG

SEQ ID NO: 104 - protein, 4 aa, synthetic construct
  REGION 1..4: note = Synthetic Construct
GGAG

SEQ ID NO: 105 - protein, 4 aa, synthetic construct
  REGION 1..4: note = Synthetic Construct
GGSG

SEQ ID NO: 106 - protein, 4 aa, synthetic construct
  REGION 1..4: note = Synthetic Construct
AGGG

SEQ ID NO: 107 - protein, 4 aa, synthetic construct
  REGION 1..4: note = Synthetic Construct
SGGG

SEQ ID NO: 108 - protein, 4 aa, synthetic construct
  REGION 1..4: note = Synthetic Construct
GAGA

SEQ ID NO: 109 - protein, 4 aa, synthetic construct
  REGION 1..4: note = Synthetic Construct
GSGS

SEQ ID NO: 110 - protein, 6 aa, synthetic construct
  REGION 1..6: note = Synthetic Construct
GAGAGA

SEQ ID NO: 111 - protein, 6 aa, synthetic construct
  REGION 1..6: note = Synthetic Construct
GSGSGS

SEQ ID NO: 112 - protein, 8 aa, synthetic construct
  REGION 1..8: note = Synthetic Construct
GAGAGAGA

SEQ ID NO: 113 - protein, 8 aa, synthetic construct
  REGION 1..8: note = Synthetic Construct
GSGSGSGS

SEQ ID NO: 114 - protein, 10 aa, synthetic construct
  REGION 1..10: note = Synthetic Construct
GAGAGAGAGA

SEQ ID NO: 115 - protein, 10 aa, synthetic construct
  REGION 1..10: note = Synthetic Construct
GSGSGSGSGS

SEQ ID NO: 116 - protein, 12 aa, synthetic construct
  REGION 1..12: note = Synthetic Construct
GAGAGAGAGAGA

SEQ ID NO: 117 - protein, 12 aa, synthetic construct
  REGION 1..12: note = Synthetic Construct
GSGSGSGSGSGS

SEQ ID NO: 118 - protein, 6 aa, synthetic construct
  REGION 1..6: note = Synthetic Construct
GGAGGA

SEQ ID NO: 119 - protein, 6 aa, synthetic construct
  REGION 1..6: note = Synthetic Construct
GGSGGS

SEQ ID NO: 120 - protein, 9 aa, synthetic construct
  REGION 1..9: note = Synthetic Construct
GGAGGAGGA

SEQ ID NO: 121 - protein, 9 aa, synthetic construct
  REGION 1..9: note = Synthetic Construct
GGSGGSGGS

SEQ ID NO: 122 - protein, 12 aa, synthetic construct
  REGION 1..12: note = Synthetic Construct
GGAGGAGGAGGA

SEQ ID NO: 123 - protein, 12 aa, synthetic construct
  REGION 1..12: note = Synthetic Construct
GGSGGSGGSGGS

SEQ ID NO: 124 - protein, 8 aa, synthetic construct
  REGION 1..8: note = Synthetic Construct
GGAGGGAG

SEQ ID NO: 125 - protein, 8 aa, synthetic construct
  REGION 1..8: note = Synthetic Construct
GGSGGGSG

SEQ ID NO: 126 - protein, 12 aa, synthetic construct
  REGION 1..12: note = Synthetic Construct
GGAGGGAGGGAG

SEQ ID NO: 127 - protein, 12 aa, synthetic construct
  REGION 1..12: note = Synthetic Construct
GGSGGGSGGGSG

SEQ ID NO: 128 - protein, 15 aa, synthetic construct
  REGION 1..15: note = Synthetic Construct
GGGGAGGGGAGGGGA

SEQ ID NO: 129 - protein, 15 aa, synthetic construct
  REGION 1..15: note = Synthetic Construct
GGGGSGGGGSGGGGS

SEQ ID NO: 130 - protein, 5 aa, synthetic construct
  REGION 1..5: note = Synthetic Construct
GGGAG

SEQ ID NO: 131 - protein, 6 aa, synthetic construct
  REGION 1..6: note = Synthetic Construct
GGGAGG

SEQ ID NO: 132 - protein, 7 aa, synthetic construct
  REGION 1..7: note = Synthetic Construct
GGGAGGG

SEQ ID NO: 133 - protein, 4 aa, synthetic construct
  REGION 1..4: note = Synthetic Construct
AAAL

SEQ ID NO: 134 - protein, 4 aa, synthetic construct
  REGION 1..4: note = Synthetic Construct
AAAK

SEQ ID NO: 135 - protein, 4 aa, synthetic construct
  REGION 1..4: note = Synthetic Construct
AAAR

SEQ ID NO: 136 - protein, 14 aa, synthetic construct
  REGION 1..14: note = Synthetic Construct
EGKSSGSGSESKST

SEQ ID NO: 137 - protein, 12 aa, synthetic construct
  REGION 1..12: note = Synthetic Construct
GSAGSAAGSGEF

SEQ ID NO: 138 - protein, 12 aa, synthetic construct
  REGION 1..12: note = Synthetic Construct
AEAAAKEAAAKA

SEQ ID NO: 139 - protein, 18 aa, synthetic construct
  REGION 1..18: note = Synthetic Construct
KESGSVSSEQLAQFRSLD

SEQ ID NO: 140 - protein, 10 aa, synthetic construct
  REGION 1..10: note = Synthetic Construct
GENLYFQSGG

SEQ ID NO: 141 - protein, 8 aa, synthetic construct
  REGION 1..8: note = Synthetic Construct
SACYCELS

SEQ ID NO: 142 - protein, 5 aa, synthetic construct
  REGION 1..5: note = Synthetic Construct
RSIAT

SEQ ID NO: 143 - protein, 17 aa, synthetic construct
  REGION 1..17: note = Synthetic Construct
RPACKIPNDLKQKVMNH

SEQ ID NO: 144 - protein, 36 aa, synthetic construct
  REGION 1..36: note = Synthetic Construct
GGSAGGSGSGSSGGSSGASGTGTAGGTGSGSGTGSG

SEQ ID NO: 145 - protein, 17 aa, synthetic construct
  REGION 1..17: note = Synthetic Construct
AAANSSIDLISVPVDSR

SEQ ID NO: 146 - protein, 36 aa, synthetic construct
  REGION 1..36: note = Synthetic Construct
GGSGGGSEGGGSEGGGSEGGGSEGGGSEGGGSGGGS

SEQ ID NO: 147 - protein, 5 aa, synthetic construct
  REGION 1..5: note = Synthetic Construct
EAAAK

SEQ ID NO: 148 - protein, 5 aa, synthetic construct
  REGION 1..5: note = Synthetic Construct
PAPAP

SEQ ID NO: 149 - protein, 109 aa, synthetic construct
  REGION 1..109: note = Synthetic Construct
GAILGRSETQECLFYNANWELERTNQTGVERCEGEKDKRLHCYATWRNISGSIEIVAKGCWLDDFNCYDRTDCVETEENPQVYFCCCEGNMCNEKFSYFPEMEVTQPTS

SEQ ID NO: 150 - protein, 227 aa, Homo sapiens
DKTHTCPPCPAPELLGGPSVFLFPPKPKDTLMISRTPEVTCVVVDVSHEDPEVKFNWYVDGVEVHNAKTKPREEQYNSTYRVVSVLTVLHQDWLNGKEYKCKVSNKALPAPIEKTISKAKGQPREPQVYTLPPSRDELTKNQVSLTCLVKGFYPSDIAVEWESNGQPENNYKTTPPVLDSDGSFFLYSKLTVDKSRWQQGNVFSCSVMHEALHNHYTQKSLSLSPGK

SEQ ID NO: 151 - protein, 11 aa, synthetic construct
  REGION 1..11: note = Synthetic Construct
DICLPRWGCLW

SEQ ID NO: 152 - protein, 93 aa, Homo sapiens
GPVEVFITETPSQPNSHPIQWNAPQPSHISKYILRWRPKNSVGRWKEATIPGHLNSYTIKGLKPGVVYEGQLISIQQYGHQEVTRFDFTTTST

SEQ ID NO: 153 - protein, 609 aa, Homo sapiens [sequence omitted]

SEQ ID NO: 154 - protein, 6 aa, synthetic construct
  REGION 1..6: note = Synthetic Construct
NPVTPK

SEQ ID NO: 155 - protein, 226 aa, Homo sapiens
DKTHTCPPCPAPELLGGPSVFLFPPKPKDTLMISRTPEVTCVVVDVSHEDPEVKFNWYVDGVEVHNAKTKPREEQYNSTYRVVSVLTVLHQDWLNGKEYKCKVSNKALPAPIEKTISKAKGQPREPQVYTLPPSRDELTKNQVSLTCLVKGFYPSDIAVEWESNGQPENNYKTTPPVLDSDGSFFLYSKLTVDKSRWQQGNVFSCSVMHEALHNHYTQKSLSLSPG

SEQ ID NO: 156 - protein, 338 aa, synthetic construct
  REGION 1..338: note = Synthetic Construct
GAILGRSETQECLFYNANWELERTNQTGVERCEGEKDKRLHCYATWRNISGSIEIVKKGCWLDDFNCYDRTDCVETEENPQVYFCCCEGNMCNEKFSYFPEMEVTQPTSGGGDKTHTCPPCPAPELLGGPSVFLFPPKPKDTLMISRTPEVTCVVVDVSHEDPEVKFNWYVDGVEVHNAKTKPREEQYNSTYRVVSVLTVLHQDWLNGKEYKCKVSNKALPAPIEKTISKAKGQPREPQVYTLPPSRDELTKNQVSLTCLVKGFYPSDIAVEWESNGQPENNYKTTPPVLDSDGSFFLYSKLTVDKSRWQQGNVFSCSVMHEALHNHYTQKSLSLSPG

SEQ ID NO: 157 - protein, 115 aa, synthetic construct
  REGION 1..115: note = Synthetic Construct
  VARIANT 11: note = MISC_FEATURE - Xaa is Ile or Leu
  VARIANT 12: note = MISC_FEATURE - Xaa is Phe or Tyr
  VARIANT 19: note = MISC_FEATURE - Xaa is Leu or Lys
  VARIANT 20: note = MISC_FEATURE - Xaa is Asp or Glu
  VARIANT 25: note = MISC_FEATURE - Xaa is Thr or Ser
  VARIANT 27: note = MISC_FEATURE - Xaa is Leu or Val
  VARIANT 29: note = MISC_FEATURE - Xaa is Pro or Arg
  VARIANT 31: note = MISC_FEATURE - Xaa is Tyr or Glu
  VARIANT 33: note = MISC_FEATURE - Xaa is Asp or Glu
  VARIANT 34: note = MISC_FEATURE - Xaa is Lys or Gln
  VARIANT 38: note = MISC_FEATURE - Xaa is Arg or Leu
  VARIANT 41: note = MISC_FEATURE - Xaa is Tyr or Phe
  VARIANT 45: note = MISC_FEATURE - Xaa is Arg or Lys
  VARIANT 47: note = MISC_FEATURE - Xaa is Ser or Ile
  VARIANT 48: note = MISC_FEATURE - Xaa is Ser or Thr
  VARIANT 50: note = MISC_FEATURE - Xaa is Ser or Thr
  VARIANT 51: note = MISC_FEATURE - Xaa is Ile or Leu
  VARIANT 53: note = MISC_FEATURE - Xaa is Ile or Leu
  VARIANT 56: note = MISC_FEATURE - Xaa is Lys or Gln
  VARIANT 63: note = MISC_FEATURE - Xaa is Phe or Ile
  VARIANT 69: note = MISC_FEATURE - Xaa is Gln, Thr, or Asp
  VARIANT 70: note = MISC_FEATURE - Xaa is Glu, Asp, or Thr
  VARIANT 74: note = MISC_FEATURE - Xaa is Lys or Thr
  VARIANT 75: note = MISC_FEATURE - Xaa is Lys or Glu
  VARIANT 76: note = MISC_FEATURE - Xaa is Asp or Glu
  VARIANT 77: note = MISC_FEATURE - Xaa is Ser or Asn
  VARIANT 79: note = MISC_FEATURE - Xaa is Glu or Gln
  VARIANT 89: note = MISC_FEATURE - Xaa is Phe or Met
GRGEAETRECXXYNANWEXXRTNQXGXEXCXGXXDKRXHCXASWXNXXGXXEXVKXGCWLDDXNCYDRXXCVAXXXXPXVYFCCCEGNXCNERFTHLPEAGGPEVTYEPPPTAPT

SEQ ID NO: 158 - protein, 115 aa, synthetic construct
  REGION 1..115: note = Synthetic Construct
GRGEAETRECIFYNANWEKDRTNQSGLEPCYGDQDKRRHCFASWKNSSGTIELVKQGCWLDDINCYDRQECVAKKDSPEVYFCCCEGNFCNERFTHLPEAGGPEVTYEPPPTAPT

SEQ ID NO: 159 - protein, 115 aa, synthetic construct
  REGION 1..115: note = Synthetic Construct
GRGEAETRECIYYNANWELDRTNQSGLERCEGEQDKRLHCYASWRNSSGTIELVKKGCWLDDINCYDRQECVATKENPQVYFCCCEGNFCNERFTHLPEAGGPEVTYEPPPTAPT

SEQ ID NO: 160 - protein, 115 aa, synthetic construct
  REGION 1..115: note = Synthetic Construct
GRGEAETRECIYYNANWELERTNQSGLERCEGEQDKRLHCYASWRNSSGTIELVKKGCWLDDFNCYDRQECVAKKDSPEVYFCCCEGNFCNERFTHLPEAGGPEVTYEPPPTAPT

SEQ ID NO: 161 - protein, 115 aa, synthetic construct
  REGION 1..115: note = Synthetic Construct
GRGEAETRECIYYNANWELERTNQTGLERCEGEQDKRLHCYASWRNISGTIELVKKGCWLDDFNCYDRQECVAKKDSPEVYFCCCEGNFCNERFTHLPEAGGPEVTYEPPPTAPT

SEQ ID NO: 162 - protein, 115 aa, synthetic construct
  REGION 1..115: note = Synthetic Construct
GRGEAETRECIYYNANWELERTNQTGLERCEGEQDKRLHCYASWRNITGTIELVKKGCWLDDFNCYDRQECVAKKDSPEVYFCCCEGNFCNERFTHLPEAGGPEVTYEPPPTAPT

SEQ ID NO: 163 - protein, 115 aa, synthetic construct
  REGION 1..115: note = Synthetic Construct
GRGEAETRECIYYNANWELERTNQSGLEPCEGEQDKRLHCYASWRNSSGTIELVKKGCWLDDFNCYDRQECVAKKDSPEVYFCCCEGNFCNERFTHLPEAGGPEVTYEPPPTAPT

SEQ ID NO: 164 - protein, 115 aa, synthetic construct
  REGION 1..115: note = Synthetic Construct
GRGEAETRECIYYNANWELERTNQSGLERCYGDKDKRLHCYASWRNSSGTIELVKKGCWLDDFNCYDRQECVAKKDSPEVYFCCCEGNFCNERFTHLPEAGGPEVTYEPPPTAPT

SEQ ID NO: 165 - protein, 115 aa, synthetic construct
  REGION 1..115: note = Synthetic Construct
GRGEAETRECIYYNANWELERTNQSGLERCEGEQDKRLHCFASWKNSSGTIELVKQGCWLDDFNCYDRQECVAKKDSPEVYFCCCEGNFCNERFTHLPEAGGPEVTYEPPPTAPT

SEQ ID NO: 166 - protein, 115 aa, synthetic construct
  REGION 1..115: note = Synthetic Construct
GRGEAETRECIFYNANWEKDRTNQSGLERCEGEQDKRLHCYASWRNSSGTIELVKKGCWLDDFNCYDRQECVAKKDSPEVYFCCCEGNFCNERFTHLPEAGGPEVTYEPPPTAPT

SEQ ID NO: 167 - protein, 115 aa, synthetic construct
  REGION 1..115: note = Synthetic Construct
GRGEAETRECIYYNANWELERTNQSGLERCYGDQDKRRHCYASWRNSSGTIELVKKGCWLDDFNCYDRQECVAKKDSPEVYFCCCEGNFCNERFTHLPEAGGPEVTYEPPPTAPT

SEQ ID NO: 168 - protein, 115 aa, synthetic construct
  REGION 1..115: note = Synthetic Construct
GRGEAETRECLYYNANWELERTNQSGVERCEGEKDKRLHCYASWRNSSGSLEIVKKGCWLDDFNCYDRTDCVATEENPQVYFCCCEGNMCNERFTHLPEAGGPEVTYEPPPTAPT

SEQ ID NO: 169 - protein, 115 aa, synthetic construct
  REGION 1..115: note = Synthetic Construct
GRGEAETRECLYYNANWELERTNQSGVERCEGEKDKRLHCYASWRNSSGSLEIVKKGCWLDDFNCYDRDTCVATEENPQVYFCCCEGNMCNERFTHLPEAGGPEVTYEPPPTAPT

SEQ ID NO: 170 - protein, 115 aa, synthetic construct
  REGION 1..115: note = Synthetic Construct
GRGEAETRECLYYNANWELERTNQSGVERCEGEKDKRLHCYASWRNSSGSLEIVKKGCWLDDFNCYDRTDCVATKENPQVYFCCCEGNMCNERFTHLPEAGGPEVTYEPPPTAPT

SEQ ID NO: 171 - protein, 115 aa, synthetic construct
  REGION 1..115: note = Synthetic Construct
GRGEAETRECLYYNANWELERTNQSGVERCEGEKDKRLHCYASWRNSSGSLEIVKKGCWLDDFNCYDRDTCVATKENPQVYFCCCEGNMCNERFTHLPEAGGPEVTYEPPPTAPT

SEQ ID NO: 172 - protein, 345 aa, synthetic construct
  REGION 1..345: note = Synthetic Construct
GRGEAETRECLYYNANWELERTNQSGVERCEGEKDKRLHCYASWRNSSGSLEIVKKGCWLDDFNCYDRDTCVATKENPQVYFCCCEGNMCNERFTHLPEAGGPEVTYEPPPTAPTGGGDKTHTCPPCPAPELLGGPSVFLFPPKPKDTLMISRTPEVTCVVVDVSHEDPEVKFNWYVDGVEVHNAKTKPREEQYNSTYRVVSVLTVLHQDWLNGKEYKCKVSNKALPAPIEKTISKAKGQPREPQVYTLPPSRDELTKNQVSLTCLVKGFYPSDIAVEWESNGQPENNYKTTPPVLDSDGSFFLYSKLTVDKSRWQQGNVFSCSVMHEALHNHYTQKSLSLSPGK

SEQ ID NO: 173 - protein, 512 aa, Homo sapiens
MTAPWVALALLWGSLCAGSGRGEAETRECIYYNANWELERTNQSGLERCEGEQDKRLHCYASWRNSSGTIELVKKGCWLDDFNCYDRQECVATEENPQVYFCCCEGNFCNERFTHLPEAGGPEVTYEPPPTAPTLLTVLAYSLLPIGGLSLIVLLAFWMYRHRKPPYGHVDIHEDPGPPPPSPLVGLKPLQLLEIKARGRFGCVWKAQLMNDFVAVKIFPLQDKQSWQSEREIFSTPGMKHENLLQFIAAEKRGSNLEVELWLITAFHDKGSLTDYLKGNIITWNELCHVAETMSRGLSYLHEDVPWCRGEGHKPSIAHRDFKSKNVLLKSDLTAVLADFGLAVRFEPGKPPGDTHGQVGTRRYMAPEVLEGAINFQRDAFLRIDMYAMGLVLWELVSRCKAADGPVDEYMLPFEEEIGQHPSLEELQEVVVHKKMRPTIKDHWLKHPGLAQLCVTIEECWDHDAEARLSAGCVEERVSLIRRSVNGTTSDCLVSLVTSVTNVDLPPKESSI

SEQ ID NO: 174 - protein, 109 aa, synthetic construct
  REGION 1..109: note = Synthetic Construct
  VARIANT 37: note = MISC_FEATURE - Xaa is Asp or Arg
  VARIANT 65: note = MISC_FEATURE - Xaa is Ile, Phe, Glu, Asp, Tyr, Ser, Asn, Gln, or Thr
  VARIANT 66: note = MISC_FEATURE - Xaa is Asn or Thr
  VARIANT 75: note = MISC_FEATURE - Xaa is Ala or Glu
  VARIANT 76: note = MISC_FEATURE - Xaa is Thr or Lys
  VARIANT 77: note = MISC_FEATURE - Xaa is Glu or Lys
  VARIANT 78: note = MISC_FEATURE - Xaa is Glu or Asp
  VARIANT 79: note = MISC_FEATURE - Xaa is Asn or Ser
  VARIANT 81: note = MISC_FEATURE - Xaa is Gln, Glu, Lys, Arg, Asp, or Asn
GAILGRAETRECIYYNANWELERTNQSGLERCEGEQXKRRHCFATWKNISGSIEIVKQGCWLDDXXCYDRTDCVXXXXXPXVYFCCCEGNMCNEKFSYFPEMEVTQPTS

SEQ ID NO: 175 - protein, 109 aa, synthetic construct
  REGION 1..109: note = Synthetic Construct
  VARIANT 37: note = MISC_FEATURE - Xaa is Asp or Arg
  VARIANT 65: note = MISC_FEATURE - Xaa is Ile, Phe, Glu, Asp, Tyr, Ser, Asn, Gln, or Thr
  VARIANT 66: note = MISC_FEATURE - Xaa is Asn or Thr
  VARIANT 75: note = MISC_FEATURE - Xaa is Ala or Glu
  VARIANT 76: note = MISC_FEATURE - Xaa is Thr or Lys
  VARIANT 77: note = MISC_FEATURE - Xaa is Glu or Lys
  VARIANT 78: note = MISC_FEATURE - Xaa is Glu or Asp
  VARIANT 79: note = MISC_FEATURE - Xaa is Asn or Ser
  VARIANT 81: note = MISC_FEATURE - Xaa is Gln, Glu, Lys, Arg, Asp, or Asn
GAILGRAETRECIYYNANWELERTNQSGLERCEGEQXKRLHCFATWKNISGSIEIVKQGCWLDDXXCYDRTDCVXXXXXPXVYFCCCEGNMCNEKFSYFPEMEVTQPTS

SEQ ID NO: 176 - protein, 109 aa, synthetic construct
  REGION 1..109: note = Synthetic Construct
  VARIANT 37: note = MISC_FEATURE - Xaa is Asp or Arg
  VARIANT 65: note = MISC_FEATURE - Xaa is Ile, Phe, Glu, Asp, Tyr, Ser, Asn, Gln, or Thr
  VARIANT 66: note = MISC_FEATURE - Xaa is Asn or Thr
  VARIANT 75: note = MISC_FEATURE - Xaa is Ala or Glu
  VARIANT 76: note = MISC_FEATURE - Xaa is Thr or Lys
  VARIANT 77: note = MISC_FEATURE - Xaa is Glu or Lys
  VARIANT 78: note = MISC_FEATURE - Xaa is Glu or Asp
  VARIANT 79: note = MISC_FEATURE - Xaa is Asn or Ser
  VARIANT 81: note = MISC_FEATURE - Xaa is Gln, Glu, Lys, Arg, Asp, or Asn
GAILGRAETRECIYYNANWELERTNQSGLERCEGEQXKRLHCYASWKNISGSIEIVKQGCWLDDXXCYDRTDCVXXXXXPXVYFCCCEGNMCNEKFSYFPEMEVTQPTS

SEQ ID NO: 177 - protein, 109 aa, synthetic construct
  REGION 1..109: note = Synthetic Construct
  VARIANT 37: note = MISC_FEATURE - Xaa is Asp or Arg
  VARIANT 65: note = MISC_FEATURE - Xaa is Ile, Phe, Glu, Asp, Tyr, Ser, Asn, Gln, or Thr
  VARIANT 66: note = MISC_FEATURE - Xaa is Asn or Thr
  VARIANT 75: note = MISC_FEATURE - Xaa is Ala or Glu
  VARIANT 76: note = MISC_FEATURE - Xaa is Thr or Lys
  VARIANT 77: note = MISC_FEATURE - Xaa is Glu or Lys
  VARIANT 78: note = MISC_FEATURE - Xaa is Glu or Asp
  VARIANT 79: note = MISC_FEATURE - Xaa is Asn or Ser
  VARIANT 81: note = MISC_FEATURE - Xaa is Gln, Glu, Lys, Arg, Asp, or Asn
GAILGRAETRECIYYNANWELERTNQSGLERCEGEQXKRLHCYASWRNSSGSIEIVKQGCWLDDXXCYDRTDCVXXXXXPXVYFCCCEGNMCNEKFSYFPEMEVTQPTS

SEQ ID NO: 178 - protein, 109 aa, synthetic construct
  REGION 1..109: note = Synthetic Construct
  VARIANT 37: note = MISC_FEATURE - Xaa is Asp or Arg
  VARIANT 65: note = MISC_FEATURE - Xaa is Ile, Phe, Glu, Asp, Tyr, Ser, Asn, Gln, or Thr
  VARIANT 66: note = MISC_FEATURE - Xaa is Asn or Thr
  VARIANT 75: note = MISC_FEATURE - Xaa is Ala or Glu
  VARIANT 76: note = MISC_FEATURE - Xaa is Thr or Lys
  VARIANT 77: note = MISC_FEATURE - Xaa is Glu or Lys
  VARIANT 78: note = MISC_FEATURE - Xaa is Glu or Asp
  VARIANT 79: note = MISC_FEATURE - Xaa is Asn or Ser
  VARIANT 81: note = MISC_FEATURE - Xaa is Gln, Glu, Lys, Arg, Asp, or Asn
GAILGRAETRECIYYNANWELERTNQSGLERCEGEQXKRLHCYASWRNSSGTIEIVKQGCWLDDXXCYDRTDCVXXXXXPXVYFCCCEGNMCNEKFSYFPEMEVTQPTS

SEQ ID NO: 179 - protein, 109 aa, synthetic construct
  REGION 1..109: note = Synthetic Construct
  VARIANT 37: note = MISC_FEATURE - Xaa is Asp or Arg
  VARIANT 65: note = MISC_FEATURE - Xaa is Ile, Phe, Glu, Asp, Tyr, Ser, Asn, Gln, or Thr
  VARIANT 66: note = MISC_FEATURE - Xaa is Asn or Thr
  VARIANT 75: note = MISC_FEATURE - Xaa is Ala or Glu
  VARIANT 76: note = MISC_FEATURE - Xaa is Thr or Lys
  VARIANT 77: note = MISC_FEATURE - Xaa is Glu or Lys
  VARIANT 78: note = MISC_FEATURE - Xaa is Glu or Asp
  VARIANT 79: note = MISC_FEATURE - Xaa is Asn or Ser
  VARIANT 81: note = MISC_FEATURE - Xaa is Gln, Glu, Lys, Arg, Asp, or Asn
GAILGRAETRECIYYNANWELERTNQSGLERCEGEQXKRLHCYASWRNSSGTIELVKKGCWLDDXXCYDRTDCVXXXXXPXVYFCCCEGNMCNEKFSYFPEMEVTQPTS

SEQ ID NO: 180 - protein, 109 aa, synthetic construct
  REGION 1..109: note = Synthetic Construct
  VARIANT 37: note = MISC_FEATURE - Xaa is Asp or Arg
  VARIANT 65: note = MISC_FEATURE - Xaa is Ile, Phe, Glu, Asp, Tyr, Ser, Asn, Gln, or Thr
  VARIANT 66: note = MISC_FEATURE - Xaa is Asn or Thr
  VARIANT 75: note = MISC_FEATURE - Xaa is Ala or Glu
  VARIANT 76: note = MISC_FEATURE - Xaa is Thr or Lys
  VARIANT 77: note = MISC_FEATURE - Xaa is Glu or Lys
  VARIANT 78: note = MISC_FEATURE - Xaa is Glu or Asp
  VARIANT 79: note = MISC_FEATURE - Xaa is Asn or Ser
  VARIANT 81: note = MISC_FEATURE - Xaa is Gln, Glu, Lys, Arg, Asp, or Asn
GAILGRAETRECIYYNANWELERTNQSGLERCEGEQXKRLHCYASWRNSSGTIELVKKGCWLDDXXCYDRQECVXXXXXPXVYFCCCEGNMCNEKFSYFPEMEVTQPTS

SEQ ID NO: 181 - protein, 107 aa, synthetic construct
  REGION 1..107: note = Synthetic Construct
  VARIANT 35: note = MISC_FEATURE - Xaa is Asp or Arg
  VARIANT 63: note = MISC_FEATURE - Xaa is Ile, Phe, Glu, Asp, Tyr, Ser, Asn, Gln, or Thr
  VARIANT 64: note = MISC_FEATURE - Xaa is Asn or Thr
  VARIANT 73: note = MISC_FEATURE - Xaa is Ala or Glu
  VARIANT 74: note = MISC_FEATURE - Xaa is Thr or Lys
  VARIANT 75: note = MISC_FEATURE - Xaa is Glu or Lys
  VARIANT 76: note = MISC_FEATURE - Xaa is Glu or Asp
  VARIANT 77: note = MISC_FEATURE - Xaa is Asn or Ser
  VARIANT 79: note = MISC_FEATURE - Xaa is Gln, Glu, Lys, Arg, Asp, or Asn
GRGEAETRECIYYNANWELERTNQSGLERCEGEQXKRRHCFATWKNISGSIEIVKQGCWLDDXXCYDRTDCVXXXXXPXVYFCCCEGNMCNEKFSYFPEMEVTQPTS

SEQ ID NO: 182 - protein, 107 aa, synthetic construct
  REGION 1..107: note = Synthetic Construct
  VARIANT 35: note = MISC_FEATURE - Xaa is Asp or Arg
  VARIANT 63: note = MISC_FEATURE - Xaa is Ile, Phe, Glu, Asp, Tyr, Ser, Asn, Gln, or Thr
  VARIANT 64: note = MISC_FEATURE - Xaa is Asn or Thr
  VARIANT 73: note = MISC_FEATURE - Xaa is Ala or Glu
  VARIANT 74: note = MISC_FEATURE - Xaa is Thr or Lys
  VARIANT 75: note = MISC_FEATURE - Xaa is Glu or Lys
  VARIANT 76: note = MISC_FEATURE - Xaa is Glu or Asp
  VARIANT 77: note = MISC_FEATURE - Xaa is Asn or Ser
  VARIANT 79: note = MISC_FEATURE - Xaa is Gln, Glu, Lys, Arg, Asp, or Asn
GRGEAETRECIYYNANWELERTNQSGLERCEGEQXKRLHCFATWKNISGSIEIVKQGCWLDDXXCYDRTDCVXXXXXPXVYFCCCEGNMCNEKFSYFPEMEVTQPTS

SEQ ID NO: 183 - protein, 107 aa, synthetic construct
  REGION 1..107: note = Synthetic Construct
  VARIANT 35: note = MISC_FEATURE - Xaa is Asp or Arg
  VARIANT 63: note = MISC_FEATURE - Xaa is Ile, Phe, Glu, Asp, Tyr, Ser, Asn, Gln, or Thr
  VARIANT 64: note = MISC_FEATURE - Xaa is Asn or Thr
  VARIANT 73: note = MISC_FEATURE - Xaa is Ala or Glu
  VARIANT 74: note = MISC_FEATURE - Xaa is Thr or Lys
  VARIANT 75: note = MISC_FEATURE - Xaa is Glu or Lys
  VARIANT 76: note = MISC_FEATURE - Xaa is Glu or Asp
  VARIANT 77: note = MISC_FEATURE - Xaa is Asn or Ser
  VARIANT 79: note = MISC_FEATURE - Xaa is Gln, Glu, Lys, Arg, Asp, or Asn
GRGEAETRECIYYNANWELERTNQSGLERCEGEQXKRLHCYASWKNISGSIEIVKQGCWLDDXXCYDRTDCVXXXXXPXVYFCCCEGNMCNEKFSYFPEMEVTQPTS

SEQ ID NO: 184 - protein, 107 aa, synthetic construct
  REGION 1..107: note = Synthetic Construct
  VARIANT 35: note = MISC_FEATURE - Xaa is Asp or Arg
  VARIANT 63: note = MISC_FEATURE - Xaa is Ile, Phe, Glu, Asp, Tyr, Ser, Asn, Gln, or Thr
  VARIANT 64: note = MISC_FEATURE - Xaa is Asn or Thr
  VARIANT 73: note = MISC_FEATURE - Xaa is Ala or Glu
  VARIANT 74: note = MISC_FEATURE - Xaa is Thr or Lys
  VARIANT 75: note = MISC_FEATURE - Xaa is Glu or Lys
  VARIANT 76: note = MISC_FEATURE - Xaa is Glu or Asp
  VARIANT 77: note = MISC_FEATURE - Xaa is Asn or Ser
  VARIANT 79: note = MISC_FEATURE - Xaa is Gln, Glu, Lys, Arg, Asp, or Asn
GRGEAETRECIYYNANWELERTNQSGLERCEGEQXKRLHCYASWRNSSGSIEIVKQGCWLDDXXCYDRTDCVXXXXXPXVYFCCCEGNMCNEKFSYFPEMEVTQPTS

SEQ ID NO: 185 - protein, 107 aa, synthetic construct
  REGION 1..107: note = Synthetic Construct
  VARIANT 35: note = MISC_FEATURE - Xaa is Asp or Arg
  VARIANT 63: note = MISC_FEATURE - Xaa is Ile, Phe, Glu, Asp, Tyr, Ser, Asn, Gln, or Thr
  VARIANT 64: note = MISC_FEATURE - Xaa is Asn or Thr
  VARIANT 73: note = MISC_FEATURE - Xaa is Ala or Glu
  VARIANT 74: note = MISC_FEATURE - Xaa is Thr or Lys
  VARIANT 75: note = MISC_FEATURE - Xaa is Glu or Lys
  VARIANT 76: note = MISC_FEATURE - Xaa is Glu or Asp
  VARIANT 77: note = MISC_FEATURE - Xaa is Asn or Ser
  VARIANT 79: note = MISC_FEATURE - Xaa is Gln, Glu, Lys, Arg, Asp, or Asn
GRGEAETRECIYYNANWELERTNQSGLERCEGEQXKRLHCYASWRNSSGTIEIVKQGCWLDDXXCYDRTDCVXXXXXPXVYFCCCEGNMCNEKFSYFPEMEVTQPTS

SEQ ID NO: 186 - protein, 107 aa, synthetic construct
  REGION 1..107: note = Synthetic Construct
  VARIANT 35: note = MISC_FEATURE - Xaa is Asp or Arg
  VARIANT 63: note = MISC_FEATURE - Xaa is Ile, Phe, Glu, Asp, Tyr, Ser, Asn, Gln, or Thr
  VARIANT 64: note = MISC_FEATURE - Xaa is Asn or Thr
  VARIANT 73: note = MISC_FEATURE - Xaa is Ala or Glu
  VARIANT 74: note = MISC_FEATURE - Xaa is Thr or Lys
  VARIANT 75: note = MISC_FEATURE - Xaa is Glu or Lys
  VARIANT 76: note = MISC_FEATURE - Xaa is Glu or Asp
  VARIANT 77: note = MISC_FEATURE - Xaa is Asn or Ser
  VARIANT 79: note = MISC_FEATURE - Xaa is Gln, Glu, Lys, Arg, Asp, or Asn
GRGEAETRECIYYNANWELERTNQSGLERCEGEQXKRLHCYASWRNSSGTIELVKKGCWLDDXXCYDRTDCVXXXXXPXVYFCCCEGNMCNEKFSYFPEMEVTQPTS

SEQ ID NO: 187 - protein, 107 aa, synthetic construct
  REGION 1..107: note = Synthetic Construct
  VARIANT 35: note = MISC_FEATURE - Xaa is Asp or Arg
  VARIANT 63: note = MISC_FEATURE - Xaa is Ile, Phe, Glu, Asp, Tyr, Ser, Asn, Gln, or Thr
  VARIANT 64: note = MISC_FEATURE - Xaa is Asn or Thr
  VARIANT 73: note = MISC_FEATURE - Xaa is Ala or Glu
  VARIANT 74: note = MISC_FEATURE - Xaa is Thr or Lys
  VARIANT 75: note = MISC_FEATURE - Xaa is Glu or Lys
  VARIANT 76: note = MISC_FEATURE - Xaa is Glu or Asp
  VARIANT 77: note = MISC_FEATURE - Xaa is Asn or Ser
  VARIANT 79: note = MISC_FEATURE - Xaa is Gln, Glu, Lys, Arg, Asp, or Asn
GRGEAETRECIYYNANWELERTNQSGLERCEGEQXKRLHCYASWRNSSGTIELVKKGCWLDDXXCYDRQECVXXXXXPXVYFCCCEGNMCNEKFSYFPEMEVTQPTS

SEQ ID NO: 188 - protein, 109 aa, synthetic construct
  REGION 1..109: note = Synthetic Construct
  VARIANT 37: note = MISC_FEATURE - Xaa is Asp or Arg
  VARIANT 65: note = MISC_FEATURE - Xaa is Ile, Phe, Glu, Asp, Tyr, Ser, Asn, Gln, or Thr
  VARIANT 66: note = MISC_FEATURE - Xaa is Asn or Thr
  VARIANT 75: note = MISC_FEATURE - Xaa is Ala or Glu
  VARIANT 76: note = MISC_FEATURE - Xaa is Thr or Lys
  VARIANT 77: note = MISC_FEATURE - Xaa is Glu or Lys
  VARIANT 78: note = MISC_FEATURE - Xaa is Glu or Asp
  VARIANT 79: note = MISC_FEATURE - Xaa is Asn or Ser
  VARIANT 81: note = MISC_FEATURE - Xaa is Gln, Glu, Lys, Arg, Asp, or Asn
GAILGRSETQECIYYNANWELERTNQSGLERCEGEQXKRRHCFATWKNISGSIEIVKQGCWLDDXXCYDRTDCVXXXXXPXVYFCCCEGNMCNEKFSYFPEMEVTQPTS

SEQ ID NO: 189 - protein, 109 aa, synthetic construct
  REGION 1..109: note = Synthetic Construct
  VARIANT 37: note = MISC_FEATURE - Xaa is Asp or Arg
  VARIANT 65: note = MISC_FEATURE - Xaa is Ile, Phe, Glu, Asp, Tyr, Ser, Asn, Gln, or Thr
  VARIANT 66: note = MISC_FEATURE - Xaa is Asn or Thr
  VARIANT 75: note = MISC_FEATURE - Xaa is Ala or Glu
  VARIANT 76: note = MISC_FEATURE - Xaa is Thr or Lys
  VARIANT 77: note = MISC_FEATURE - Xaa is Glu or Lys
  VARIANT 78: note = MISC_FEATURE - Xaa is Glu or Asp
  VARIANT 79: note = MISC_FEATURE - Xaa is Asn or Ser
  VARIANT 81: note = MISC_FEATURE - Xaa is Gln, Glu, Lys, Arg, Asp, or Asn
GAILGRSETQECIYYNANWELERTNQSGLERCEGEQXKRLHCFATWKNISGSIEIVKQGCWLDDXXCYDRTDCVXXXXXPXVYFCCCEGNMCNEKFSYFPEMEVTQPTS

SEQ ID NO: 190 - protein, 109 aa, synthetic construct
  REGION 1..109: note = Synthetic Construct
  VARIANT 37: note = MISC_FEATURE - Xaa is Asp or Arg
  VARIANT 65: note = MISC_FEATURE - Xaa is Ile, Phe, Glu, Asp, Tyr, Ser, Asn, Gln, or Thr
  VARIANT 66: note = MISC_FEATURE - Xaa is Asn or Thr
  VARIANT 75: note = MISC_FEATURE - Xaa is Ala or Glu
  VARIANT 76: note = MISC_FEATURE - Xaa is Thr or Lys
  VARIANT 77: note = MISC_FEATURE - Xaa is Glu or Lys
  VARIANT 78: note = MISC_FEATURE - Xaa is Glu or Asp
  VARIANT 79: note = MISC_FEATURE - Xaa is Asn or Ser
  VARIANT 81: note = MISC_FEATURE - Xaa is Gln, Glu, Lys, Arg, Asp, or Asn
GAILGRSETQECIYYNANWELERTNQSGLERCEGEQXKRLHCYASWKNISGSIEIVKQGCWLDDXXCYDRTDCVXXXXXPXVYFCCCEGNMCNEKFSYFPEMEVTQPTS

SEQ ID NO: 191 - protein, 109 aa, synthetic construct
  REGION 1..109: note = Synthetic Construct
  VARIANT 37: note = MISC_FEATURE - Xaa is Asp or Arg
  VARIANT 65: note = MISC_FEATURE - Xaa is Ile, Phe, Glu, Asp, Tyr, Ser, Asn, Gln, or Thr
  VARIANT 66: note = MISC_FEATURE - Xaa is Asn or Thr
  VARIANT 75: note = MISC_FEATURE - Xaa is Ala or Glu
  VARIANT 76: note = MISC_FEATURE - Xaa is Thr or Lys
  VARIANT 77: note = MISC_FEATURE - Xaa is Glu or Lys
  VARIANT 78: note = MISC_FEATURE - Xaa is Glu or Asp
  VARIANT 79: note = MISC_FEATURE - Xaa is Asn or Ser
  VARIANT 81: note = MISC_FEATURE - Xaa is Gln, Glu, Lys, Arg, Asp, or Asn
GAILGRSETQECIYYNANWELERTNQSGLERCEGEQXKRLHCYASWRNSSGSIEIVKQGCWLDDXXCYDRTDCVXXXXXPXVYFCCCEGNMCNEKFSYFPEMEVTQPTS

SEQ ID NO: 192 - protein, 109 aa, synthetic construct
  REGION 1..109: note = Synthetic Construct
  VARIANT 37: note = MISC_FEATURE - Xaa is Asp or Arg
  VARIANT 65: note = MISC_FEATURE - Xaa is Ile, Phe, Glu, Asp, Tyr, Ser, Asn, Gln, or Thr
  VARIANT 66: note = MISC_FEATURE - Xaa is Asn or Thr
  VARIANT 75: note = MISC_FEATURE - Xaa is Ala or Glu
  VARIANT 76: note = MISC_FEATURE - Xaa is Thr or Lys
  VARIANT 77: note = MISC_FEATURE - Xaa is Glu or Lys
  VARIANT 78: note = MISC_FEATURE - Xaa is Glu or Asp
  VARIANT 79: note = MISC_FEATURE - Xaa is Asn or Ser
  VARIANT 81: note = MISC_FEATURE - Xaa is Gln, Glu, Lys, Arg, Asp, or Asn
GAILGRSETQECIYYNANWELERTNQSGLERCEGEQXKRLHCYASWRNSSGTIEIVKQGCWLDDXXCYDRTDCVXXXXXPXVYFCCCEGNMCNEKFSYFPEMEVTQPTS

SEQ ID NO: 193 - protein, 109 aa, synthetic construct
  REGION 1..109: note = Synthetic Construct
  VARIANT 37: note = MISC_FEATURE - Xaa is Asp or Arg
  VARIANT 65: note = MISC_FEATURE - Xaa is Ile, Phe, Glu, Asp, Tyr, Ser, Asn, Gln, or Thr
  VARIANT 66: note = MISC_FEATURE - Xaa is Asn or Thr
  VARIANT 75: note = MISC_FEATURE - Xaa is Ala or Glu
  VARIANT 76: note = MISC_FEATURE - Xaa is Thr or Lys
  VARIANT 77: note = MISC_FEATURE - Xaa is Glu or Lys
  VARIANT 78: note = MISC_FEATURE - Xaa is Glu or Asp
  VARIANT 79: note = MISC_FEATURE - Xaa is Asn or Ser
  VARIANT 81: note = MISC_FEATURE - Xaa is Gln, Glu, Lys, Arg, Asp, or Asn
GAILGRSETQECIYYNANWELERTNQSGLERCEGEQXKRLHCYASWRNSSGTIELVKKGCWLDDXXCYDRTDCVXXXXXPXVYFCCCEGNMCNEKFSYFPEMEVTQPTS

SEQ ID NO: 194 - protein, 109 aa, synthetic construct
  REGION 1..109: note = Synthetic Construct
  VARIANT 37: note = MISC_FEATURE - Xaa is Asp or Arg
  VARIANT 65: note = MISC_FEATURE - Xaa is Ile, Phe, Glu, Asp, Tyr, Ser, Asn, Gln, or Thr
  VARIANT 66: note = MISC_FEATURE - Xaa is Asn or Thr
  VARIANT 75: note = MISC_FEATURE - Xaa is Ala or Glu
  VARIANT 76: note = MISC_FEATURE - Xaa is Thr or Lys
  VARIANT 77: note = MISC_FEATURE - Xaa is Glu or Lys
  VARIANT 78: note = MISC_FEATURE - Xaa is Glu or Asp
  VARIANT 79: note = MISC_FEATURE - Xaa is Asn or Ser
  VARIANT 81: note = MISC_FEATURE - Xaa is Gln, Glu, Lys, Arg, Asp, or Asn
GAILGRSETQECIYYNANWELERTNQSGLERCEGEQXKRLHCYASWRNSSGTIELVKKGCWLDDXXCYDRQECVXXXXXPXVYFCCCEGNMCNEKFSYFPEMEVTQPTS

SEQ ID NO: 195 - protein, 109 aa, synthetic construct
  REGION 1..109: note = Synthetic Construct
GAILGRAETRECIYYNANWELERTNQSGLERCEGEQDKRLHCYASWRNSSGTIEIVKQGCWLDDINCYDRTDCVATEENPQVYFCCCEGNMCNEKFSYFPEMEVTQPTS

SEQ ID NO: 196 - protein, 107 aa, synthetic construct
  REGION 1..107: note = Synthetic Construct
GRGEAETRECIYYNANWELERTNQSGLERCEGEQDKRLHCYASWRNSSGTIEIVKQGCWLDDINCYDRTDCVEKKDSPEVYFCCCEGNMCNEKFSYFPEMEVTQPTS

SEQ ID NO: 197 - protein, 107 aa, synthetic construct
  REGION 1..107: note = Synthetic Construct
GRGEAETRECIYYNANWELERTNQSGLERCEGEQDKRLHCYASWRNSSGTIEIVKQGCWLDDINCYDRTDCVEKKDSPQVYFCCCEGNMCNEKFSYFPEMEVTQPTS

SEQ ID NO: 198 - protein, 107 aa, synthetic construct
  REGION 1..107: note = Synthetic Construct
GRGEAETRECIYYNANWELERTNQSGLERCEGEQDKRLHCYASWRNSSGTIEIVKQGCWLDDFNCYDRTDCVEKKDSPQVYFCCCEGNMCNEKFSYFPEMEVTQPTS

SEQ ID NO: 199 - protein, 109 aa, synthetic construct
  REGION 1..109: note = Synthetic Construct
GAILGRAETRECIYYNANWELERTNQSGLERCEGEQDKRLHCYASWRNSSGTIEIVKQGCWLDDFNCYDRTDCVATEENPQVYFCCCEGNMCNEKFSYFPEMEVTQPTS

SEQ ID NO: 200 - protein, 107 aa, synthetic construct
  REGION 1..107: note = Synthetic Construct
GRGEAETRECIYYNANWELERTNQSGLERCEGEQDKRLHCYASWRNSSGTIEIVKQGCWLDDFNCYDRTDCVEKKDSPEVYFCCCEGNMCNEKFSYFPEMEVTQPTS

SEQ ID NO: 201 - protein, 107 aa, synthetic construct
  REGION 1..107: note = Synthetic Construct
GRGEAETRECIYYNANWELERTNQSGLERCEGEQDKRRHCFATWKNISGSIEIVKQGCWLDDFNCYDRTDCVEKKDSPQVYFCCCEGNMCNEKFSYFPEMEVTQPTS

SEQ ID NO: 202 - protein, 107 aa, synthetic construct
  REGION 1..107: note = Synthetic Construct
GRGEAETRECIYYNANWELERTNQSGLERCEGEQDKRLHCFATWKNISGSIEIVKQGCWLDDFNCYDRTDCVEKKDSPQVYFCCCEGNMCNEKFSYFPEMEVTQPTS

SEQ ID NO: 203 - protein, 107 aa, synthetic construct
  REGION 1..107: note = Synthetic Construct
GRGEAETRECIYYNANWELERTNQSGLERCEGEQDKRLHCYASWKNISGSIEIVKQGCWLDDFNCYDRTDCVEKKDSPQVYFCCCEGNMCNEKFSYFPEMEVTQPTS

SEQ ID NO: 204 - protein, 107 aa, synthetic construct
  REGION 1..107: note = Synthetic Construct
GRGEAETRECIYYNANWELERTNQSGLERCEGEQDKRLHCYASWRNSSGSIEIVKQGCWLDDFNCYDRTDCVEKKDSPQVYFCCCEGNMCNEKFSYFPEMEVTQPTS

SEQ ID NO: 205 - protein, 107 aa, synthetic construct
  REGION 1..107: note = Synthetic Construct
GRGEAETRECIYYNANWELERTNQSGLERCEGEQDKRLHCYASWRNSSGTIELVKKGCWLDDFNCYDRTDCVEKKDSPQVYFCCCEGNMCNEKFSYFPEMEVTQPTS

SEQ ID NO: 206 - protein, 107 aa, synthetic construct
  REGION 1..107: note = Synthetic Construct
GRGEAETRECIYYNANWELERTNQSGLERCEGEQDKRLHCYASWRNSSGTIELVKKGCWLDDFNCYDRQECVATKDSPQVYFCCCEGNMCNEKFSYFPEMEVTQPTS

SEQ ID NO: 207 - protein, 107 aa, synthetic construct
  REGION 1..107: note = Synthetic Construct
GRGEAETRECIYYNANWELERTNQSGLERCEGEQDKRLHCYASWRNSSGTIELVKKGCWLDDFNCYDRQECVATEENPQVYFCCCEGNMCNEKFSYFPEMEVTQPTS

SEQ ID NO: 208 - protein, 107 aa, synthetic construct
  REGION 1..107: note = Synthetic Construct
GRGEAETRECIYYNANWELERTNQSGLERCEGEQDKRLHCYASWRNSSGTIEIVKQGCWLDDNNCYDRTDCVEKKDSPQVYFCCCEGNMCNEKFSYFPEMEVTQPTS

SEQ ID NO: 209 - protein, 107 aa, synthetic construct
  REGION 1..107: note = Synthetic Construct
GRGEAETRECIYYNANWELERTNQSGLERCEGEQDKRLHCYASWRNSSGTIEIVKQGCWLDDTNCYDRTDCVEKKDSPQVYFCCCEGNMCNEKFSYFPEMEVTQPTS

SEQ ID NO: 210 - protein, 107 aa, synthetic construct
  REGION 1..107: note = Synthetic Construct
GRGEAETRECIYYNANWELERTNQSGLERCEGEQDKRLHCYASWRNSSGTIEIVKQGCWLDDETCYDRTDCVEKKDSPQVYFCCCEGNMCNEKFSYFPEMEVTQPTS

SEQ ID NO: 211 - protein, 107 aa, synthetic construct
  REGION 1..107: note = Synthetic Construct
GRGEAETRECIYYNANWELERTNQSGLERCEGEQRKRLHCYASWRNSSGTIEIVKQGCWLDDFNCYDRTDCVEKKDSPQVYFCCCEGNMCNEKFSYFPEMEVTQPTS

SEQ ID NO: 212 - protein, 107 aa, synthetic construct
  REGION 1..107: note = Synthetic Construct
GRGEAETRECIYYNANWELERTNQSGLERCEGEQDKRLHCYASWRNSSGTIEIVKQGCWLDDFNCYDRTDCVETKDSPQVYFCCCEGNMCNEKFSYFPEMEVTQPTS

SEQ ID NO: 213 - protein, 109 aa, synthetic construct
  REGION 1..109: note = Synthetic Construct
GAILGRAETRECIYYNANWELERTNQSGLERCEGEQDKRLHCYASWRNSSGTIEIVKQGCWLDDFNCYDRTDCVEKKDSPQVYFCCCEGNMCNEKFSYFPEMEVTQPTS

SEQ ID NO: 214 - protein, 109 aa, synthetic construct
  REGION 1..109: note = Synthetic Construct
GAILGRSETQECIYYNANWELERTNQSGLERCEGEQDKRLHCYASWRNSSGTIEIVKQGCWLDDFNCYDRTDCVEKKDSPQVYFCCCEGNMCNEKFSYFPEMEVTQPTS

SEQ ID NO: 215 - protein, 107 aa, synthetic construct
  REGION 1..107: note = Synthetic Construct
GRGEAETRECIYYNANWELERTNQSGLERCEGEQDKRLHCYASWRNSSGTIELVKKGCWLDDFNCYDRQECVATKDSPEVYFCCCEGNMCNEKFSYFPEMEVTQPTS

SEQ ID NO: 216 - protein, 107 aa, synthetic construct
  REGION 1..107: note = Synthetic Construct
GRGEAETRECIYYNANWELERTNQSGLERCEGEQDKRLHCYASWRNSSGTIELVKKGCWLDDFNCYDRQECVATKENPQVYFCCCEGNMCNEKFSYFPEMEVTQPTS

SEQ ID NO: 217 - protein, 339 aa, synthetic construct
  REGION 1..339: note = Synthetic Construct
GAILGRAETRECIYYNANWELERTNQSGLERCEGEQDKRLHCYASWRNSSGTIEIVKQGCWLDDINCYDRTDCVATEENPQVYFCCCEGNMCNEKFSYFPEMEVTQPTSGGGDKTHTCPPCPAPELLGGPSVFLFPPKPKDTLMISRTPEVTCVVVDVSHEDPEVKFNWYVDGVEVHNAKTKPREEQYNSTYRVVSVLTVLHQDWLNGKEYKCKVSNKALPAPIEKTISKAKGQPREPQVYTLPPSRDELTKNQVSLTCLVKGFYPSDIAVEWESNGQPENNYKTTPPVLDSDGSFFLYSKLTVDKSRWQQGNVFSCSVMHEALHNHYTQKSLSLSPGK

SEQ ID NO: 218 - protein, 337 aa, synthetic construct
  REGION 1..337: note = Synthetic Construct
GRGEAETRECIYYNANWELERTNQSGLERCEGEQDKRLHCYASWRNSSGTIEIVKQGCWLDDINCYDRTDCVEKKDSPEVYFCCCEGNMCNEKFSYFPEMEVTQPTSGGGDKTHTCPPCPAPELLGGPSVFLFPPKPKDTLMISRTPEVTCVVVDVSHEDPEVKFNWYVDGVEVHNAKTKPREEQYNSTYRVVSVLTVLHQDWLNGKEYKCKVSNKALPAPIEKTISKAKGQPREPQVYTLPPSRDELTKNQVSLTCLVKGFYPSDIAVEWESNGQPENNYKTTPPVLDSDGSFFLYSKLTVDKSRWQQGNVFSCSVMHEALHNHYTQKSLSLSPGK

SEQ ID NO: 219 - protein, 337 aa, synthetic construct
  REGION 1..337: note = Synthetic Construct
GRGEAETRECIYYNANWELERTNQSGLERCEGEQDKRLHCYASWRNSSGTIEIVKQGCWLDDINCYDRTDCVEKKDSPQVYFCCCEGNMCNEKFSYFPEMEVTQPTSGGGDKTHTCPPCPAPELLGGPSVFLFPPKPKDTLMISRTPEVTCVVVDVSHEDPEVKFNWYVDGVEVHNAKTKPREEQYNSTYRVVSVLTVLHQDWLNGKEYKCKVSNKALPAPIEKTISKAKGQPREPQVYTLPPSRDELTKNQVSLTCLVKGFYPSDIAVEWESNGQPENNYKTTPPVLDSDGSFFLYSKLTVDKSRWQQGNVFSCSVMHEALHNHYTQKSLSLSPGK

SEQ ID NO: 220 - protein, 337 aa, synthetic construct
  REGION 1..337: note = Synthetic Construct
GRGEAETRECIYYNANWELERTNQSGLERCEGEQDKRLHCYASWRNSSGTIEIVKQGCWLDDFNCYDRTDCVEKKDSPQVYFCCCEGNMCNEKFSYFPEMEVTQPTSGGGDKTHTCPPCPAPELLGGPSVFLFPPKPKDTLMISRTPEVTCVVVDVSHEDPEVKFNWYVDGVEVHNAKTKPREEQYNSTYRVVSVLTVLHQDWLNGKEYKCKVSNKALPAPIEKTISKAKGQPREPQVYTLPPSRDELTKNQVSLTCLVKGFYPSDIAVEWESNGQPENNYKTTPPVLDSDGSFFLYSKLTVDKSRWQQGNVFSCSVMHEALHNHYTQKSLSLSPGK

SEQ ID NO: 221 - protein, 107 aa, synthetic construct
  REGION 1..107: note = Synthetic Construct
ILGRAETRECIYYNANWELERTNQSGLERCEGEQDKRLHCYASWRNSSGTIEIVKQGCWLDDINCYDRTDCVATEENPQVYFCCCEGNMCNEKFSYFPEMEVTQPTS

SEQ ID NO: 222 - protein, 106 aa, synthetic construct
  REGION 1..106: note = Synthetic Construct
RGEAETRECIYYNANWELERTNQSGLERCEGEQDKRLHCYASWRNSSGTIEIVKQGCWLDDINCYDRTDCVEKKDSPEVYFCCCEGNMCNEKFSYFPEMEVTQPTS

SEQ ID NO: 223 - protein, 106 aa, synthetic construct
  REGION 1..106: note = Synthetic Construct
RGEAETRECIYYNANWELERTNQSGLERCEGEQDKRLHCYASWRNSSGTIEIVKQGCWLDDINCYDRTDCVEKKDSPQVYFCCCEGNMCNEKFSYFPEMEVTQPTS

SEQ ID NO: 224 - protein, 106 aa, synthetic construct
  REGION 1..106: note = Synthetic Construct
RGEAETRECIYYNANWELERTNQSGLERCEGEQDKRLHCYASWRNSSGTIEIVKQGCWLDDFNCYDRTDCVEKKDSPQVYFCCCEGNMCNEKFSYFPEMEVTQPTS

SEQ ID NO: 225 - protein, 106 aa, synthetic construct
  REGION 1..106: note = Synthetic Construct
LGRAETRECIYYNANWELERTNQSGLERCEGEQDKRLHCYASWRNSSGTIEIVKQGCWLDDINCYDRTDCVATEENPQVYFCCCEGNMCNEKFSYFPEMEVTQPTS

SEQ ID NO: 226 - protein, 105 aa, synthetic construct
  REGION 1..105: note = Synthetic Construct
GEAETRECIYYNANWELERTNQSGLERCEGEQDKRLHCYASWRNSSGTIEIVKQGCWLDDINCYDRTDCVEKKDSPEVYFCCCEGNMCNEKFSYFPEMEVTQPTS

SEQ ID NO: 227 - protein, 105 aa, synthetic construct
  REGION 1..105: note = Synthetic Construct
GEAETRECIYYNANWELERTNQSGLERCEGEQDKRLHCYASWRNSSGTIEIVKQGCWLDDINCYDRTDCVEKKDSPQVYFCCCEGNMCNEKFSYFPEMEVTQPTS

SEQ ID NO: 228 - protein, 105 aa, synthetic construct
  REGION 1..105: note = Synthetic Construct
GEAETRECIYYNANWELERTNQSGLERCEGEQDKRLHCYASWRNSSGTIEIVKQGCWLDDFNCYDRTDCVEKKDSPQVYFCCCEGNMCNEKFSYFPEMEVTQPTS

SEQ ID NO: 229 - protein, 105 aa, synthetic construct
  REGION 1..105: note = Synthetic Construct
GRAETRECIYYNANWELERTNQSGLERCEGEQDKRLHCYASWRNSSGTIEIVKQGCWLDDINCYDRTDCVATEENPQVYFCCCEGNMCNEKFSYFPEMEVTQPTS

SEQ ID NO: 230 - protein, 104 aa, synthetic construct
  REGION 1..104: note = Synthetic Construct
EAETRECIYYNANWELERTNQSGLERCEGEQDKRLHCYASWRNSSGTIEIVKQGCWLDDINCYDRTDCVEKKDSPEVYFCCCEGNMCNEKFSYFPEMEVTQPTS

SEQ ID NO: 231 - protein, 104 aa, synthetic construct
  REGION 1..104: note = Synthetic Construct
EAETRECIYYNANWELERTNQSGLERCEGEQDKRLHCYASWRNSSGTIEIVKQGCWLDDINCYDRTDCVEKKDSPQVYFCCCEGNMCNEKFSYFPEMEVTQPTS

SEQ ID NO: 232 - protein, 104 aa, synthetic construct
  REGION 1..104: note = Synthetic Construct
EAETRECIYYNANWELERTNQSGLERCEGEQDKRLHCYASWRNSSGTIEIVKQGCWLDDFNCYDRTDCVEKKDSPQVYFCCCEGNMCNEKFSYFPEMEVTQPTS

SEQ ID NO: 233 - protein, 104 aa, synthetic construct
  REGION 1..104: note = Synthetic Construct
RAETRECIYYNANWELERTNQSGLERCEGEQDKRLHCYASWRNSSGTIEIVKQGCWLDDINCYDRTDCVATEENPQVYFCCCEGNMCNEKFSYFPEMEVTQPTS

SEQ ID NO: 234 - protein, 103 aa, synthetic construct
  REGION 1..103: note = Synthetic Construct
AETRECIYYNANWELERTNQSGLERCEGEQDKRLHCYASWRNSSGTIEIVKQGCWLDDINCYDRTDCVEKKDSPEVYFCCCEGNMCNEKFSYFPEMEVTQPTS

SEQ ID NO: 235 - protein, 103 aa, synthetic construct
  REGION 1..103: note = Synthetic Construct
AETRECIYYNANWELERTNQSGLERCEGEQDKRLHCYASWRNSSGTIEIVKQGCWLDDINCYDRTDCVEKKDSPQVYFCCCEGNMCNEKFSYFPEMEVTQPTS

SEQ ID NO: 236 - protein, 103 aa, synthetic construct
  REGION 1..103: note = Synthetic Construct
AETRECIYYNANWELERTNQSGLERCEGEQDKRLHCYASWRNSSGTIEIVKQGCWLDDFNCYDRTDCVEKKDSPQVYFCCCEGNMCNEKFSYFPEMEVTQPTS

SEQ ID NO: 237 - protein, 103 aa, synthetic construct
  REGION 1..103: note = Synthetic Construct
AETRECIYYNANWELERTNQSGLERCEGEQDKRLHCYASWRNSSGTIEIVKQGCWLDDINCYDRTDCVATEENPQVYFCCCEGNMCNEKFSYFPEMEVTQPTS

SEQ ID NO: 238 - protein, 102 aa, synthetic construct
  REGION 1..102: note = Synthetic Construct
ETRECIYYNANWELERTNQSGLERCEGEQDKRLHCYASWRNSSGTIEIVKQGCWLDDINCYDRTDCVEKKDSPEVYFCCCEGNMCNEKFSYFPEMEVTQPTS

SEQ ID NO: 239 - protein, 102 aa, synthetic construct
  REGION 1..102: note = Synthetic Construct
ETRECIYYNANWELERTNQSGLERCEGEQDKRLHCYASWRNSSGTIEIVKQGCWLDDINCYDRTDCVEKKDSPQVYFCCCEGNMCNEKFSYFPEMEVTQPTS

SEQ ID NO: 240 - protein, 102 aa, synthetic construct
  REGION 1..102: note = Synthetic Construct
ETRECIYYNANWELERTNQSGLERCEGEQDKRLHCYASWRNSSGTIEIVKQGCWLDDFNCYDRTDCVEKKDSPQVYFCCCEGNMCNEKFSYFPEMEVTQPTS

SEQ ID NO: 241 - protein, 102 aa, synthetic construct
  REGION 1..102: note = Synthetic Construct
ETRECIYYNANWELERTNQSGLERCEGEQDKRLHCYASWRNSSGTIEIVKQGCWLDDINCYDRTDCVATEENPQVYFCCCEGNMCNEKFSYFPEMEVTQPTS

SEQ ID NO: 242 - protein, 101 aa, synthetic construct
  REGION 1..101: note = Synthetic Construct
TRECIYYNANWELERTNQSGLERCEGEQDKRLHCYASWRNSSGTIEIVKQGCWLDDINCYDRTDCVEKKDSPEVYFCCCEGNMCNEKFSYFPEMEVTQPTS

SEQ ID NO: 243 - protein, 101 aa, synthetic construct
  REGION 1..101: note = Synthetic Construct
TRECIYYNANWELERTNQSGLERCEGEQDKRLHCYASWRNSSGTIEIVKQGCWLDDINCYDRTDCVEKKDSPQVYFCCCEGNMCNEKFSYFPEMEVTQPTS

SEQ ID NO: 244 - protein, 101 aa, synthetic construct
  REGION 1..101: note = Synthetic Construct
TRECIYYNANWELERTNQSGLERCEGEQDKRLHCYASWRNSSGTIEIVKQGCWLDDFNCYDRTDCVEKKDSPQVYFCCCEGNMCNEKFSYFPEMEVTQPTS

SEQ ID NO: 245 - protein, 101 aa, synthetic construct
  REGION 1..101: note = Synthetic Construct
TRECIYYNANWELERTNQSGLERCEGEQDKRLHCYASWRNSSGTIEIVKQGCWLDDINCYDRTDCVATEENPQVYFCCCEGNMCNEKFSYFPEMEVTQPTS

SEQ ID NO: 246 - protein, 100 aa, synthetic construct
  REGION 1..100: note = Synthetic Construct
RECIYYNANWELERTNQSGLERCEGEQDKRLHCYASWRNSSGTIEIVKQGCWLDDINCYDRTDCVEKKDSPEVYFCCCEGNMCNEKFSYFPEMEVTQPTS

SEQ ID NO: 247 - protein, 100 aa, synthetic construct
  REGION 1..100: note = Synthetic Construct
RECIYYNANWELERTNQSGLERCEGEQDKRLHCYASWRNSSGTIEIVKQGCWLDDINCYDRTDCVEKKDSPQVYFCCCEGNMCNEKFSYFPEMEVTQPTS

SEQ ID NO: 248 - protein, 100 aa, synthetic construct
  REGION 1..100: note = Synthetic Construct
RECIYYNANWELERTNQSGLERCEGEQDKRLHCYASWRNSSGTIEIVKQGCWLDDFNCYDRTDCVEKKDSPQVYFCCCEGNMCNEKFSYFPEMEVTQPTS

SEQ ID NO: 249 - protein, 100 aa, synthetic construct
  REGION 1..100: note = Synthetic Construct
RECIYYNANWELERTNQSGLERCEGEQDKRLHCYASWRNSSGTIEIVKQGCWLDDINCYDRTDCVATEENPQVYFCCCEGNMCNEKFSYFPEMEVTQPTS

SEQ ID NO: 250 - protein, 106 aa, synthetic construct
  REGION 1..106: note = Synthetic Construct
RGEAETRECIYYNANWELERTNQSGLERCEGEQDKRRHCFATWKNISGSIEIVKQGCWLDDFNCYDRTDCVEKKDSPQVYFCCCEGNMCNEKFSYFPEMEVTQPTS

SEQ ID NO: 251 - protein, 106 aa, synthetic construct
  REGION 1..106: note = Synthetic Construct
RGEAETRECIYYNANWELERTNQSGLERCEGEQDKRLHCYASWRNSSGTIEIVKQGCWLDDETCYDRTDCVEKKDSPQVYFCCCEGNMCNEKFSYFPEMEVTQPTS

SEQ ID NO: 252 - protein, 107 aa, synthetic construct
  REGION 1..107: note = Synthetic Construct
ILGRAETRECIYYNANWELERTNQSGLERCEGEQDKRLHCYASWRNSSGTIEIVKQGCWLDDFNCYDRTDCVEKKDSPQVYFCCCEGNMCNEKFSYFPEMEVTQPTS

SEQ ID NO: 253 - protein, 107 aa, synthetic construct
  REGION 1..107: note = Synthetic Construct
ILGRSETQECIYYNANWELERTNQSGLERCEGEQDKRLHCYASWRNSSGTIEIVKQGCWLDDFNCYDRTDCVEKKDSPQVYFCCCEGNMCNEKFSYFPEMEVTQPTS

SEQ ID NO: 254 - protein, 106 aa, synthetic construct
  REGION 1..106: note = Synthetic Construct
RGEAETRECIYYNANWELERTNQSGLERCEGEQDKRLHCYASWRNSSGTIELVKKGCWLDDFNCYDRQECVATKDSPEVYFCCCEGNMCNEKFSYFPEMEVTQPTS

SEQ ID NO: 255 - protein, 106 aa, synthetic construct
  REGION 1..106: note = Synthetic Construct
RGEAETRECIYYNANWELERTNQSGLERCEGEQDKRLHCYASWRNSSGTIELVKKGCWLDDFNCYDRQECVATKENPQVYFCCCEGNMCNEKFSYFPEMEVTQPTS

SEQ ID NO: 256 - protein, 105 aa, synthetic construct
  REGION 1..105: note = Synthetic Construct
GEAETRECIYYNANWELERTNQSGLERCEGEQDKRRHCFATWKNISGSIEIVKQGCWLDDFNCYDRTDCVEKKDSPQVYFCCCEGNMCNEKFSYFPEMEVTQPTS

SEQ ID NO: 257 - protein, 105 aa, synthetic construct
  REGION 1..105: note = Synthetic Construct
GEAETRECIYYNANWELERTNQSGLERCEGEQDKRLHCYASWRNSSGTIEIVKQGCWLDDETCYDRTDCVEKKDSPQVYFCCCEGNMCNEKFSYFPEMEVTQPTS

SEQ ID NO: 258 - protein, 106 aa, synthetic construct
  REGION 1..106: note = Synthetic Construct
LGRAETRECIYYNANWELERTNQSGLERCEGEQDKRLHCYASWRNSSGTIEIVKQGCWLDDFNCYDRTDCVEKKDSPQVYFCCCEGNMCNEKFSYFPEMEVTQPTS

SEQ ID NO: 259 - protein, 106 aa, synthetic construct
  REGION 1..106: note = Synthetic Construct
LGRSETQECIYYNANWELERTNQSGLERCEGEQDKRLHCYASWRNSSGTIEIVKQGCWLDDFNCYDRTDCVEKKDSPQVYFCCCEGNMCNEKFSYFPEMEVTQPTS

SEQ ID NO: 260 - protein, 105 aa, synthetic construct
  REGION 1..105: note = Synthetic Construct
GEAETRECIYYNANWELERTNQSGLERCEGEQDKRLHCYASWRNSSGTIELVKKGCWLDDFNCYDRQECVATKDSPEVYFCCCEGNMCNEKFSYFPEMEVTQPTS

SEQ ID NO: 261 - protein, 105 aa, synthetic construct
  REGION 1..105: note = Synthetic Construct
GEAETRECIYYNANWELERTNQSGLERCEGEQDKRLHCYASWRNSSGTIELVKKGCWLDDFNCYDRQECVATKENPQVYFCCCEGNMCNEKFSYFPEMEVTQPTS

SEQ ID NO: 262 - protein, 104 aa, synthetic construct
  REGION 1..104: note = Synthetic Construct
EAETRECIYYNANWELERTNQSGLERCEGEQDKRRHCFATWKNISGSIEIVKQGCWLDDFNCYDRTDCVEKKDSPQVYFCCCEGNMCNEKFSYFPEMEVTQPTS

SEQ ID NO: 263 - protein, 104 aa, synthetic construct
  REGION 1..104: note = Synthetic Construct
EAETRECIYYNANWELERTNQSGLERCEGEQDKRLHCYASWRNSSGTIEIVKQGCWLDDETCYDRTDCVEKKDSPQVYFCCCEGNMCNEKFSYFPEMEVTQPTS

SEQ ID NO: 264 - protein, 105 aa, synthetic construct
  REGION 1..105: note = Synthetic Construct
GRAETRECIYYNANWELERTNQSGLERCEGEQDKRLHCYASWRNSSGTIEIVKQGCWLDDFNCYDRTDCVEKKDSPQVYFCCCEGNMCNEKFSYFPEMEVTQPTS

SEQ ID NO: 265 - protein, 105 aa, synthetic construct
  REGION 1..105: note = Synthetic Construct
GRSETQECIYYNANWELERTNQSGLERCEGEQDKRLHCYASWRNSSGTIEIVKQGCWLDDFNCYDRTDCVEKKDSPQVYFCCCEGNMCNEKFSYFPEMEVTQPTS

SEQ ID NO: 266 - protein, 104 aa, synthetic construct
  REGION 1..104: note = Synthetic Construct
EAETRECIYYNANWELERTNQSGLERCEGEQDKRLHCYASWRNSSGTIELVKKGCWLDDFNCYDRQECVATKDSPEVYFCCCEGNMCNEKFSYFPEMEVTQPTS

SEQ ID NO: 267 - protein, 104 aa, synthetic construct
  REGION 1..104: note = Synthetic Construct
EAETRECIYYNANWELERTNQSGLERCEGEQDKRLHCYASWRNSSGTIELVKKGCWLDDFNCYDRQECVATKENPQVYFCCCEGNMCNEKFSYFPEMEVTQPTS

SEQ ID NO: 268 - protein, 103 aa, synthetic construct
  REGION 1..103: note = Synthetic Construct
AETRECIYYNANWELERTNQSGLERCEGEQDKRRHCFATWKNISGSIEIVKQGCWLDDFNCYDRTDCVEKKDSPQVYFCCCEGNMCNEKFSYFPEMEVTQPTS

SEQ ID NO: 269 - protein, 103 aa, synthetic construct
  REGION 1..103: note = Synthetic Construct
AETRECIYYNANWELERTNQSGLERCEGEQDKRLHCYASWRNSSGTIEIVKQGCWLDDETCYDRTDCVEKKDSPQVYFCCCEGNMCNEKFSYFPEMEVTQPTS

SEQ ID NO: 270 - protein, 104 aa, synthetic construct
  REGION 1..104: note = Synthetic Construct
RAETRECIYYNANWELERTNQSGLERCEGEQDKRLHCYASWRNSSGTIEIVKQGCWLDDFNCYDRTDCVEKKDSPQVYFCCCEGNMCNEKFSYFPEMEVTQPTS

SEQ ID NO: 271 - protein, 104 aa, synthetic construct
  REGION 1..104: note = Synthetic Construct
RSETQECIYYNANWELERTNQSGLERCEGEQDKRLHCYASWRNSSGTIEIVKQGCWLDDFNCYDRTDCVEKKDSPQVYFCCCEGNMCNEKFSYFPEMEVTQPTS

SEQ ID NO: 272 - protein, 103 aa, synthetic construct
  REGION 1..103: note = Synthetic Construct
AETRECIYYNANWELERTNQSGLERCEGEQDKRLHCYASWRNSSGTIELVKKGCWLDDFNCYDRQECVATKDSPEVYFCCCEGNMCNEKFSYFPEMEVTQPTS

SEQ ID NO: 273 - protein, 103 aa, synthetic construct
  REGION 1..103: note = Synthetic Construct
AETRECIYYNANWELERTNQSGLERCEGEQDKRLHCYASWRNSSGTIELVKKGCWLDDFNCYDRQECVATKENPQVYFCCCEGNMCNEKFSYFPEMEVTQPTS

SEQ ID NO: 274 - protein, 102 aa, synthetic construct
  REGION 1..102: note = Synthetic Construct
ETRECIYYNANWELERTNQSGLERCEGEQDKRRHCFATWKNISGSIEIVKQGCWLDDFNCYDRTDCVEKKDSPQVYFCCCEGNMCNEKFSYFPEMEVTQPTS

SEQ ID NO: 275 - protein, 102 aa, synthetic construct
  REGION 1..102: note = Synthetic Construct
ETRECIYYNANWELERTNQSGLERCEGEQDKRLHCYASWRNSSGTIEIVKQGCWLDDETCYDRTDCVEKKDSPQVYFCCCEGNMCNEKFSYFPEMEVTQPTS

SEQ ID NO: 276 - protein, 103 aa, synthetic construct; identical to SEQ ID NO: 236
  REGION 1..103: note = Synthetic Construct

SEQ ID NO: 277 - protein, 103 aa, synthetic construct
  REGION 1..103: note = Synthetic Construct
SETQECIYYNANWELERTNQSGLERCEGEQDKRLHCYASWRNSSGTIEIVKQGCWLDDFNCYDRTDCVEKKDSPQVYFCCCEGNMCNEKFSYFPEMEVTQPTS

SEQ ID NO: 278 - protein, 102 aa, synthetic construct
  REGION 1..102: note = Synthetic Construct
ETRECIYYNANWELERTNQSGLERCEGEQDKRLHCYASWRNSSGTIELVKKGCWLDDFNCYDRQECVATKDSPEVYFCCCEGNMCNEKFSYFPEMEVTQPTS

SEQ ID NO: 279 - protein, 102 aa, synthetic construct
  REGION 1..102: note = Synthetic Construct
ETRECIYYNANWELERTNQSGLERCEGEQDKRLHCYASWRNSSGTIELVKKGCWLDDFNCYDRQECVATKENPQVYFCCCEGNMCNEKFSYFPEMEVTQPTS

SEQ ID NO: 280 - protein, 101 aa, synthetic construct
  REGION 1..101: note = Synthetic Construct
TRECIYYNANWELERTNQSGLERCEGEQDKRRHCFATWKNISGSIEIVKQGCWLDDFNCYDRTDCVEKKDSPQVYFCCCEGNMCNEKFSYFPEMEVTQPTS

SEQ ID NO: 281 - protein, 101 aa, synthetic construct
  REGION 1..101: note = Synthetic Construct
TRECIYYNANWELERTNQSGLERCEGEQDKRLHCYASWRNSSGTIEIVKQGCWLDDETCYDRTDCVEKKDSPQVYFCCCEGNMCNEKFSYFPEMEVTQPTS

SEQ ID NO: 282 - protein, 102 aa, synthetic construct; identical to SEQ ID NO: 240
  REGION 1..102: note = Synthetic Construct

SEQ ID NO: 283 - protein, 102 aa, synthetic construct
  REGION 1..102: note = Synthetic Construct
ETQECIYYNANWELERTNQSGLERCEGEQDKRLHCYASWRNSSGTIEIVKQGCWLDDFNCYDRTDCVEKKDSPQVYFCCCEGNMCNEKFSYFPEMEVTQPTS

SEQ ID NO: 284 - protein, 101 aa, synthetic construct
  REGION 1..101: note = Synthetic Construct
TRECIYYNANWELERTNQSGLERCEGEQDKRLHCYASWRNSSGTIELVKKGCWLDDFNCYDRQECVATKDSPEVYFCCCEGNMCNEKFSYFPEMEVTQPTS

SEQ ID NO: 285 - protein, 101 aa, synthetic construct
  REGION 1..101: note = Synthetic Construct
TRECIYYNANWELERTNQSGLERCEGEQDKRLHCYASWRNSSGTIELVKKGCWLDDFNCYDRQECVATKENPQVYFCCCEGNMCNEKFSYFPEMEVTQPTS

SEQ ID NO: 286 - protein, 100 aa, synthetic construct
  REGION 1..100: note = Synthetic Construct
RECIYYNANWELERTNQSGLERCEGEQDKRRHCFATWKNISGSIEIVKQGCWLDDFNCYDRTDCVEKKDSPQVYFCCCEGNMCNEKFSYFPEMEVTQPTS

SEQ ID NO: 287 - protein, 100 aa, synthetic construct
  REGION 1..100: note = Synthetic Construct
RECIYYNANWELERTNQSGLERCEGEQDKRLHCYASWRNSSGTIEIVKQGCWLDDETCYDRTDCVEKKDSPQVYFCCCEGNMCNEKFSYFPEMEVTQPTS

SEQ ID NO: 288 - protein, 101 aa, synthetic construct; identical to SEQ ID NO: 244
  REGION 1..101: note = Synthetic Construct

SEQ ID NO: 289 - protein, 101 aa, synthetic construct
  REGION 1..101: note = Synthetic Construct
TQECIYYNANWELERTNQSGLERCEGEQDKRLHCYASWRNSSGTIEIVKQGCWLDDFNCYDRTDCVEKKDSPQVYFCCCEGNMCNEKFSYFPEMEVTQPTS

SEQ ID NO: 290 - protein, 100 aa, synthetic construct
  REGION 1..100: note = Synthetic Construct
RECIYYNANWELERTNQSGLERCEGEQDKRLHCYASWRNSSGTIELVKKGCWLDDFNCYDRQECVATKDSPEVYFCCCEGNMCNEKFSYFPEMEVTQPTS

SEQ ID NO: 291 - protein, 100 aa, synthetic construct
  REGION 1..100: note = Synthetic Construct
RECIYYNANWELERTNQSGLERCEGEQDKRLHCYASWRNSSGTIELVKKGCWLDDFNCYDRQECVATKENPQVYFCCCEGNMCNEKFSYFPEMEVTQPTS

SEQ ID NO: 292 - protein, 100 aa, synthetic construct; identical to SEQ ID NO: 248
  REGION 1..100: note = Synthetic Construct

SEQ ID NO: 293 - protein, 100 aa, synthetic construct
  REGION 1..100: note = Synthetic Construct
QECIYYNANWELERTNQSGLERCEGEQDKRLHCYASWRNSSGTIEIVKQGCWLDDFNCYDRTDCVEKKDSPQVYFCCCEGNMCNEKFSYFPEMEVTQPTS

SEQ ID NO: 294 - protein, 337 aa, synthetic construct
  REGION 1..337: note = Synthetic Construct
ILGRAETRECIYYNANWELERTNQSGLERCEGEQDKRLHCYASWRNSSGTIEIVKQGCWLDDINCYDRTDCVATEENPQVYFCCCEGNMCNEKFSYFPEMEVTQPTSGGGDKTHTCPPCPAPELLGGPSVFLFPPKPKDTLMISRTPEVTCVVVDVSHEDPEVKFNWYVDGVEVHNAKTKPREEQYNSTYRVVSVLTVLHQDWLNGKEYKCKVSNKALPAPIEKTISKAKGQPREPQVYTLPPSRDELTKNQVSLTCLVKGFYPSDIAVEWESNGQPENNYKTTPPVLDSDGSFFLYSKLTVDKSRWQQGNVFSCSVMHEALHNHYTQKSLSLSPGK

SEQ ID NO: 295 - protein, 336 aa, synthetic construct
  REGION 1..336: note = Synthetic Construct
RGEAETRECIYYNANWELERTNQSGLERCEGEQDKRLHCYASWRNSSGTIEIVKQGCWLDDINCYDRTDCVEKKDSPEVYFCCCEGNMCNEKFSYFPEMEVTQPTSGGGDKTHTCPPCPAPELLGGPSVFLFPPKPKDTLMISRTPEVTCVVVDVSHEDPEVKFNWYVDGVEVHNAKTKPREEQYNSTYRVVSVLTVLHQDWLNGKEYKCKVSNKALPAPIEKTISKAKGQPREPQVYTLPPSRDELTKNQVSLTCLVKGFYPSDIAVEWESNGQPENNYKTTPPVLDSDGSFFLYSKLTVDKSRWQQGNVFSCSVMHEALHNHYTQKSLSLSPGK

SEQ ID NO: 296 - protein, 336 aa, synthetic construct
  REGION 1..336: note = Synthetic Construct
RGEAETRECIYYNANWELERTNQSGLERCEGEQDKRLHCYASWRNSSGTIEIVKQGCWLDDINCYDRTDCVEKKDSPQVYFCCCEGNMCNEKFSYFPEMEVTQPTSGGGDKTHTCPPCPAPELLGGPSVFLFPPKPKDTLMISRTPEVTCVVVDVSHEDPEVKFNWYVDGVEVHNAKTKPREEQYNSTYRVVSVLTVLHQDWLNGKEYKCKVSNKALPAPIEKTISKAKGQPREPQVYTLPPSRDELTKNQVSLTCLVKGFYPSDIAVEWESNGQPENNYKTTPPVLDSDGSFFLYSKLTVDKSRWQQGNVFSCSVMHEALHNHYTQKSLSLSPGK

SEQ ID NO: 297 - protein, 336 aa, synthetic construct
  REGION 1..336: note = Synthetic Construct
RGEAETRECIYYNANWELERTNQSGLERCEGEQDKRLHCYASWRNSSGTIEIVKQGCWLDDFNCYDRTDCVEKKDSPQVYFCCCEGNMCNEKFSYFPEMEVTQPTSGGGDKTHTCPPCPAPELLGGPSVFLFPPKPKDTLMISRTPEVTCVVVDVSHEDPEVKFNWYVDGVEVHNAKTKPREEQYNSTYRVVSVLTVLHQDWLNGKEYKCKVSNKALPAPIEKTISKAKGQPREPQVYTLPPSRDELTKNQVSLTCLVKGFYPSDIAVEWESNGQPENNYKTTPPVLDSDGSFFLYSKLTVDKSRWQQGNVFSCSVMHEALHNHYTQKSLSLSPGK

SEQ ID NO: 298 - protein, 336 aa, synthetic construct
  REGION 1..336: note = Synthetic Construct
LGRAETRECIYYNANWELERTNQSGLERCEGEQDKRLHCYASWRNSSGTIEIVKQGCWLDDINCYDRTDCVATEENPQVYFCCCEGNMCNEKFSYFPEMEVTQPTSGGGDKTHTCPPCPAPELLGGPSVFLFPPKPKDTLMISRTPEVTCVVVDVSHEDPEVKFNWYVDGVEVHNAKTKPREEQYNSTYRVVSVLTVLHQDWLNGKEYKCKVSNKALPAPIEKTISKAKGQPREPQVYTLPPSRDELTKNQVSLTCLVKGFYPSDIAVEWESNGQPENNYKTTPPVLDSDGSFFLYSKLTVDKSRWQQGNVFSCSVMHEALHNHYTQKSLSLSPGK

SEQ ID NO: 299 - protein, 335 aa, synthetic construct
  REGION 1..335: note = Synthetic Construct
GEAETRECIYYNANWELERTNQSGLERCEGEQDKRLHCYASWRNSSGTIEIVKQGCWLDDINCYDRTDCVEKKDSPEVYFCCCEGNMCNEKFSYFPEMEVTQPTSGGGDKTHTCPPCPAPELLGGPSVFLFPPKPKDTLMISRTPEVTCVVVDVSHEDPEVKFNWYVDGVEVHNAKTKPREEQYNSTYRVVSVLTVLHQDWLNGKEYKCKVSNKALPAPIEKTISKAKGQPREPQVYTLPPSRDELTKNQVSLTCLVKGFYPSDIAVEWESNGQPENNYKTTPPVLDSDGSFFLYSKLTVDKSRWQQGNVFSCSVMHEALHNHYTQKSLSLSPGK

SEQ ID NO: 300 - protein, 335 aa, synthetic construct
  REGION 1..335: note = Synthetic Construct
GEAETRECIYYNANWELERTNQSGLERCEGEQDKRLHCYASWRNSSGTIEIVKQGCWLDDINCYDRTDCVEKKDSPQVYFCCCEGNMCNEKFSYFPEMEVTQPTSGGGDKTHTCPPCPAPELLGGPSVFLFPPKPKDTLMISRTPEVTCVVVDVSHEDPEVKFNWYVDGVEVHNAKTKPREEQYNSTYRVVSVLTVLHQDWLNGKEYKCKVSNKALPAPIEKTISKAKGQPREPQVYTLPPSRDELTKNQVSLTCLVKGFYPSDIAVEWESNGQPENNYKTTPPVLDSDGSFFLYSKLTVDKSRWQQGNVFSCSVMHEALHNHYTQKSLSLSPGK

SEQ ID NO: 301 - protein, 335 aa, synthetic construct
  REGION 1..335: note = Synthetic Construct
GEAETRECIYYNANWELERTNQSGLERCEGEQDKRLHCYASWRNSSGTIEIVKQGCWLDDFNCYDRTDCVEKKDSPQVYFCCCEGNMCNEKFSYFPEMEVTQPTSGGGDKTHTCPPCPAPELLGGPSVFLFPPKPKDTLMISRTPEVTCVVVDVSHEDPEVKFNWYVDGVEVHNAKTKPREEQYNSTYRVVSVLTVLHQDWLNGKEYKCKVSNKALPAPIEKTISKAKGQPREPQVYTLPPSRDELTKNQVSLTCLVKGFYPSDIAVEWESNGQPENNYKTTPPVLDSDGSFFLYSKLTVDKSRWQQGNVFSCSVMHEALHNHYTQKSLSLSPGK

SEQ ID NO: 302 - protein, 335 aa, synthetic construct
  REGION 1..335: note = Synthetic Construct
GRAETRECIYYNANWELERTNQSGLERCEGEQDKRLHCYASWRNSSGTIEIVKQGCWLDDINCYDRTDCVATEENPQVYFCCCEGNMCNEKFSYFPEMEVTQPTSGGGDKTHTCPPCPAPELLGGPSVFLFPPKPKDTLMISRTPEVTCVVVDVSHEDPEVKFNWYVDGVEVHNAKTKPREEQYNSTYRVVSVLTVLHQDWLNGKEYKCKVSNKALPAPIEKTISKAKGQPREPQVYTLPPSRDELTKNQVSLTCLVKGFYPSDIAVEWESNGQPENNYKTTPPVLDSDGSFFLYSKLTVDKSRWQQGNVFSCSVMHEALHNHYTQKSLSLSPGK

SEQ ID NO: 303 - protein, 334 aa, synthetic construct
  REGION 1..334: note = Synthetic Construct
EAETRECIYYNANWELERTNQSGLERCEGEQDKRLHCYASWRNSSGTIEIVKQGCWLDDINCYDRTDCVEKKDSPEVYFCCCEGNMCNEKFSYFPEMEVTQPTSGGGDKTHTCPPCPAPELLGGPSVFLFPPKPKDTLMISRTPEVTCVVVDVSHEDPEVKFNWYVDGVEVHNAKTKPREEQYNSTYRVVSVLTVLHQDWLNGKEYKCKVSNKALPAPIEKTISKAKGQPREPQVYTLPPSRDELTKNQVSLTCLVKGFYPSDIAVEWESNGQPENNYKTTPPVLDSDGSFFLYSKLTVDKSRWQQGNVFSCSVMHEALHNHYTQKSLSLSPGK

SEQ ID NO: 304 - protein, 334 aa, synthetic construct
  REGION 1..334: note = Synthetic Construct
EAETRECIYYNANWELERTNQSGLERCEGEQDKRLHCYASWRNSSGTIEIVKQGCWLDDINCYDRTDCVEKKDSPQVYFCCCEGNMCNEKFSYFPEMEVTQPTSGGGDKTHTCPPCPAPELLGGPSVFLFPPKPKDTLMISRTPEVTCVVVDVSHEDPEVKFNWYVDGVEVHNAKTKPREEQYNSTYRVVSVLTVLHQDWLNGKEYKCKVSNKALPAPIEKTISKAKGQPREPQVYTLPPSRDELTKNQVSLTCLVKGFYPSDIAVEWESNGQPENNYKTTPPVLDSDGSFFLYSKLTVDKSRWQQGNVFSCSVMHEALHNHYTQKSLSLSPGK

SEQ ID NO: 305 - protein, 334 aa, synthetic construct
  REGION 1..334: note = Synthetic Construct
EAETRECIYYNANWELERTNQSGLERCEGEQDKRLHCYASWRNSSGTIEIVKQGCWLDDFNCYDRTDCVEKKDSPQVYFCCCEGNMCNEKFSYFPEMEVTQPTSGGGDKTHTCPPCPAPELLGGPSVFLFPPKPKDTLMISRTPEVTCVVVDVSHEDPEVKFNWYVDGVEVHNAKTKPREEQYNSTYRVVSVLTVLHQDWLNGKEYKCKVSNKALPAPIEKTISKAKGQPREPQVYTLPPSRDELTKNQVSLTCLVKGFYPSDIAVEWESNGQPENNYKTTPPVLDSDGSFFLYSKLTVDKSRWQQGNVFSCSVMHEALHNHYTQKSLSLSPGK

SEQ ID NO: 306 - protein, 334 aa, synthetic construct
  REGION 1..334: note = Synthetic Construct
RAETRECIYYNANWELERTNQSGLERCEGEQDKRLHCYASWRNSSGTIEIVKQGCWLDDINCYDRTDCVATEENPQVYFCCCEGNMCNEKFSYFPEMEVTQPTSGGGDKTHTCPPCPAPELLGGPSVFLFPPKPKDTLMISRTPEVTCVVVDVSHEDPEVKFNWYVDGVEVHNAKTKPREEQYNSTYRVVSVLTVLHQDWLNGKEYKCKVSNKALPAPIEKTISKAKGQPREPQVYTLPPSRDELTKNQVSLTCLVKGFYPSDIAVEWESNGQPENNYKTTPPVLDSDGSFFLYSKLTVDKSRWQQGNVFSCSVMHEALHNHYTQKSLSLSPGK

SEQ ID NO: 307 - protein, 333 aa, synthetic construct
  REGION 1..333: note = Synthetic Construct
AETRECIYYNANWELERTNQSGLERCEGEQDKRLHCYASWRNSSGTIEIVKQGCWLDDINCYDRTDCVEKKDSPEVYFCCCEGNMCNEKFSYFPEMEVTQPTSGGGDKTHTCPPCPAPELLGGPSVFLFPPKPKDTLMISRTPEVTCVVVDVSHEDPEVKFNWYVDGVEVHNAKTKPREEQYNSTYRVVSVLTVLHQDWLNGKEYKCKVSNKALPAPIEKTISKAKGQPREPQVYTLPPSRDELTKNQVSLTCLVKGFYPSDIAVEWESNGQPENNYKTTPPVLDSDGSFFLYSKLTVDKSRWQQGNVFSCSVMHEALHNHYTQKSLSLSPGK

SEQ ID NO: 308 - protein, 333 aa, synthetic construct
  REGION 1..333: note = Synthetic Construct
AETRECIYYNANWELERTNQSGLERCEGEQDKRLHCYASWRNSSGTIEIVKQGCWLDDINCYDRTDCVEKKDSPQVYFCCCEGNMCNEKFSYFPEMEVTQPTSGGGDKTHTCPPCPAPELLGGPSVFLFPPKPKDTLMISRTPEVTCVVVDVSHEDPEVKFNWYVDGVEVHNAKTKPREEQYNSTYRVVSVLTVLHQDWLNGKEYKCKVSNKALPAPIEKTISKAKGQPREPQVYTLPPSRDELTKNQVSLTCLVKGFYPSDIAVEWESNGQPENNYKTTPPVLDSDGSFFLYSKLTVDKSRWQQGNVFSCSVMHEALHNHYTQKSLSLSPGK

SEQ ID NO: 309 - protein, 333 aa, synthetic construct
  REGION 1..333: note = Synthetic Construct
AETRECIYYNANWELERTNQSGLERCEGEQDKRLHCYASWRNSSGTIEIVKQGCWLDDFNCYDRTDCVEKKDSPQVYFCCCEGNMCNEKFSYFPEMEVTQPTSGGGDKTHTCPPCPAPELLGGPSVFLFPPKPKDTLMISRTPEVTCVVVDVSHEDPEVKFNWYVDGVEVHNAKTKPREEQYNSTYRVVSVLTVLHQDWLNGKEYKCKVSNKALPAPIEKTISKAKGQPREPQVYTLPPSRDELTKNQVSLTCLVKGFYPSDIAVEWESNGQPENNYKTTPPVLDSDGSFFLYSKLTVDKSRWQQGNVFSCSVMHEALHNHYTQKSLSLSPGK

SEQ ID NO: 310 - protein, 333 aa, synthetic construct
  REGION 1..333: note = Synthetic Construct
AETRECIYYNANWELERTNQSGLERCEGEQDKRLHCYASWRNSSGTIEIVKQGCWLDDINCYDRTDCVATEENPQVYFCCCEGNMCNEKFSYFPEMEVTQPTSGGGDKTHTCPPCPAPELLGGPSVFLFPPKPKDTLMISRTPEVTCVVVDVSHEDPEVKFNWYVDGVEVHNAKTKPREEQYNSTYRVVSVLTVLHQDWLNGKEYKCKVSNKALPAPIEKTISKAKGQPREPQVYTLPPSRDELTKNQVSLTCLVKGFYPSDIAVEWESNGQPENNYKTTPPVLDSDGSFFLYSKLTVDKSRWQQGNVFSCSVMHEALHNHYTQKSLSLSPGK

SEQ ID NO: 311 - protein, 332 aa, synthetic construct
  REGION 1..332: note = Synthetic Construct
ETRECIYYNANWELERTNQSGLERCEGEQDKRLHCYASWRNSSGTIEIVKQGCWLDDINCYDRTDCVEKKDSPEVYFCCCEGNMCNEKFSYFPEMEVTQPTSGGGDKTHTCPPCPAPELLGGPSVFLFPPKPKDTLMISRTPEVTCVVVDVSHEDPEVKFNWYVDGVEVHNAKTKPREEQYNSTYRVVSVLTVLHQDWLNGKEYKCKVSNKALPAPIEKTISKAKGQPREPQVYTLPPSRDELTKNQVSLTCLVKGFYPSDIAVEWESNGQPENNYKTTPPVLDSDGSFFLYSKLTVDKSRWQQGNVFSCSVMHEALHNHYTQKSLSLSPGK

SEQ ID NO: 312 - protein, 332 aa, synthetic construct
  REGION 1..332: note = Synthetic Construct
ETRECIYYNANWELERTNQSGLERCEGEQDKRLHCYASWRNSSGTIEIVKQGCWLDDINCYDRTDCVEKKDSPQVYFCCCEGNMCNEKFSYFPEMEVTQPTSGGGDKTHTCPPCPAPELLGGPSVFLFPPKPKDTLMISRTPEVTCVVVDVSHEDPEVKFNWYVDGVEVHNAKTKPREEQYNSTYRVVSVLTVLHQDWLNGKEYKCKVSNKALPAPIEKTISKAKGQPREPQVYTLPPSRDELTKNQVSLTCLVKGFYPSDIAVEWESNGQPENNYKTTPPVLDSDGSFFLYSKLTVDKSRWQQGNVFSCSVMHEALHNHYTQKSLSLSPGK

SEQ ID NO: 313 - protein, 332 aa, synthetic construct
  REGION 1..332: note = Synthetic Construct
ETRECIYYNANWELERTNQSGLERCEGEQDKRLHCYASWRNSSGTIEIVKQGCWLDDFNCYDRTDCVEKKDSPQVYFCCCEGNMCNEKFSYFPEMEVTQPTSGGGDKTHTCPPCPAPELLGGPSVFLFPPKPKDTLMISRTPEVTCVVVDVSHEDPEVKFNWYVDGVEVHNAKTKPREEQYNSTYRVVSVLTVLHQDWLNGKEYKCKVSNKALPAPIEKTISKAKGQPREPQVYTLPPSRDELTKNQVSLTCLVKGFYPSDIAVEWESNGQPENNYKTTPPVLDSDGSFFLYSKLTVDKSRWQQGNVFSCSVMHEALHNHYTQKSLSLSPGK

SEQ ID NO: 314 - protein, 332 aa, synthetic construct
  REGION 1..332: note = Synthetic Construct
ETRECIYYNANWELERTNQSGLERCEGEQDKRLHCYASWRNSSGTIEIVKQGCWLDDINCYDRTDCVATEENPQVYFCCCEGNMCNEKFSYFPEMEVTQPTSGGGDKTHTCPPCPAPELLGGPSVFLFPPKPKDTLMISRTPEVTCVVVDVSHEDPEVKFNWYVDGVEVHNAKTKPREEQYNSTYRVVSVLTVLHQDWLNGKEYKCKVSNKALPAPIEKTISKAKGQPREPQVYTLPPSRDELTKNQVSLTCLVKGFYPSDIAVEWESNGQPENNYKTTPPVLDSDGSFFLYSKLTVDKSRWQQGNVFSCSVMHEALHNHYTQKSLSLSPGK

SEQ ID NO: 315 - protein, 331 aa, synthetic construct
  REGION 1..331: note = Synthetic Construct
TRECIYYNANWELERTNQSGLERCEGEQDKRLHCYASWRNSSGTIEIVKQGCWLDDINCYDRTDCVEKKDSPEVYFCCCEGNMCNEKFSYFPEMEVTQPTSGGGDKTHTCPPCPAPELLGGPSVFLFPPKPKDTLMISRTPEVTCVVVDVSHEDPEVKFNWYVDGVEVHNAKTKPREEQYNSTYRVVSVLTVLHQDWLNGKEYKCKVSNKALPAPIEKTISKAKGQPREPQVYTLPPSRDELTKNQVSLTCLVKGFYPSDIAVEWESNGQPENNYKTTPPVLDSDGSFFLYSKLTVDKSRWQQGNVFSCSVMHEALHNHYTQKSLSLSPGK

SEQ ID NO: 316 - protein, 331 aa, synthetic construct
  REGION 1..331: note = Synthetic Construct
TRECIYYNANWELERTNQSGLERCEGEQDKRLHCYASWRNSSGTIEIVKQGCWLDDINCYDRTDCVEKKDSPQVYFCCCEGNMCNEKFSYFPEMEVTQPTSGGGDKTHTCPPCPAPELLGGPSVFLFPPKPKDTLMISRTPEVTCVVVDVSHEDPEVKFNWYVDGVEVHNAKTKPREEQYNSTYRVVSVLTVLHQDWLNGKEYKCKVSNKALPAPIEKTISKAKGQPREPQVYTLPPSRDELTKNQVSLTCLVKGFYPSDIAVEWESNGQPENNYKTTPPVLDSDGSFFLYSKLTVDKSRWQQGNVFSCSVMHEALHNHYTQKSLSLSPGK

SEQ ID NO: 317 - protein, 331 aa, synthetic construct
  REGION 1..331: note = Synthetic Construct
TRECIYYNANWELERTNQSGLERCEGEQDKRLHCYASWRNSSGTIEIVKQGCWLDDFNCYDRTDCVEKKDSPQVYFCCCEGNMCNEKFSYFPEMEVTQPTSGGGDKTHTCPPCPAPELLGGPSVFLFPPKPKDTLMISRTPEVTCVVVDVSHEDPEVKFNWYVDGVEVHNAKTKPREEQYNSTYRVVSVLTVLHQDWLNGKEYKCKVSNKALPAPIEKTISKAKGQPREPQVYTLPPSRDELTKNQVSLTCLVKGFYPSDIAVEWESNGQPENNYKTTPPVLDSDGSFFLYSKLTVDKSRWQQGNVFSCSVMHEALHNHYTQKSLSLSPGK

SEQ ID NO: 318 - protein, 331 aa, synthetic construct
  REGION 1..331: note = Synthetic Construct
TRECIYYNANWELERTNQSGLERCEGEQDKRLHCYASWRNSSGTIEIVKQGCWLDDINCYDRTDCVATEENPQVYFCCCEGNMCNEKFSYFPEMEVTQPTSGGGDKTHTCPPCPAPELLGGPSVFLFPPKPKDTLMISRTPEVTCVVVDVSHEDPEVKFNWYVDGVEVHNAKTKPREEQYNSTYRVVSVLTVLHQDWLNGKEYKCKVSNKALPAPIEKTISKAKGQPREPQVYTLPPSRDELTKNQVSLTCLVKGFYPSDIAVEWESNGQPENNYKTTPPVLDSDGSFFLYSKLTVDKSRWQQGNVFSCSVMHEALHNHYTQKSLSLSPGK

SEQ ID NO: 319 - protein, 330 aa, synthetic construct
  REGION 1..330: note = Synthetic Construct
RECIYYNANWELERTNQSGLERCEGEQDKRLHCYASWRNSSGTIEIVKQGCWLDDINCYDRTDCVEKKDSPEVYFCCCEGNMCNEKFSYFPEMEVTQPTSGGGDKTHTCPPCPAPELLGGPSVFLFPPKPKDTLMISRTPEVTCVVVDVSHEDPEVKFNWYVDGVEVHNAKTKPREEQYNSTYRVVSVLTVLHQDWLNGKEYKCKVSNKALPAPIEKTISKAKGQPREPQVYTLPPSRDELTKNQVSLTCLVKGFYPSDIAVEWESNGQPENNYKTTPPVLDSDGSFFLYSKLTVDKSRWQQGNVFSCSVMHEALHNHYTQKSLSLSPGK

SEQ ID NO: 320 - protein, 330 aa, synthetic construct
  REGION 1..330: note = Synthetic Construct
RECIYYNANWELERTNQSGLERCEGEQDKRLHCYASWRNSSGTIEIVKQGCWLDDINCYDRTDCVEKKDSPQVYFCCCEGNMCNEKFSYFPEMEVTQPTSGGGDKTHTCPPCPAPELLGGPSVFLFPPKPKDTLMISRTPEVTCVVVDVSHEDPEVKFNWYVDGVEVHNAKTKPREEQYNSTYRVVSVLTVLHQDWLNGKEYKCKVSNKALPAPIEKTISKAKGQPREPQVYTLPPSRDELTKNQVSLTCLVKGFYPSDIAVEWESNGQPENNYKTTPPVLDSDGSFFLYSKLTVDKSRWQQGNVFSCSVMHEALHNHYTQKSLSLSPGK

SEQ ID NO: 321 - protein, 330 aa, synthetic construct
  REGION 1..330: note = Synthetic Construct
RECIYYNANWELERTNQSGLERCEGEQDKRLHCYASWRNSSGTIEIVKQGCWLDDFNCYDRTDCVEKKDSPQVYFCCCEGNMCNEKFSYFPEMEVTQPTSGGGDKTHTCPPCPAPELLGGPSVFLFPPKPKDTLMISRTPEVTCVVVDVSHEDPEVKFNWYVDGVEVHNAKTKPREEQYNSTYRVVSVLTVLHQDWLNGKEYKCKVSNKALPAPIEKTISKAKGQPREPQVYTLPPSRDELTKNQVSLTCLVKGFYPSDIAVEWESNGQPENNYKTTPPVLDSDGSFFLYSKLTVDKSRWQQGNVFSCSVMHEALHNHYTQKSLSLSPGK

SEQ ID NO: 322 - protein, 330 aa, synthetic construct
  REGION 1..330: note = Synthetic Construct
RECIYYNANWELERTNQSGLERCEGEQDKRLHCYASWRNSSGTIEIVKQGCWLDDINCYDRTDCVATEENPQVYFCCCEGNMCNEKFSYFPEMEVTQPTSGGGDKTHTCPPCPAPELLGGPSVFLFPPKPKDTLMISRTPEVTCVVVDVSHEDPEVKFNWYVDGVEVHNAKTKPREEQYNSTYRVVSVLTVLHQDWLNGKEYKCKVSNKALPAPIEKTISKAKGQPREPQVYTLPPSRDELTKNQVSLTCLVKGFYPSDIAVEWESNGQPENNYKTTPPVLDSDGSFFLYSKLTVDKSRWQQGNVFSCSVMHEALHNHYTQKSLSLSPGK

SEQ ID NO: 323 - protein, 337 aa, synthetic construct
  REGION 1..337: note = Synthetic Construct
GRGEAETRECIYYNANWELERTNQSGLERCEGEQDKRRHCFATWKNISGSIEIVKQGCWLDDFNCYDRTDCVEKKDSPQVYFCCCEGNMCNEKFSYFPEMEVTQPTSGGGDKTHTCPPCPAPELLGGPSVFLFPPKPKDTLMISRTPEVTCVVVDVSHEDPEVKFNWYVDGVEVHNAKTKPREEQYNSTYRVVSVLTVLHQDWLNGKEYKCKVSNKALPAPIEKTISKAKGQPREPQVYTLPPSRDELTKNQVSLTCLVKGFYPSDIAVEWESNGQPENNYKTTPPVLDSDGSFFLYSKLTVDKSRWQQGNVFSCSVMHEALHNHYTQKSLSLSPGK

SEQ ID NO: 324 - protein, 337 aa, synthetic construct
  REGION 1..337: note = Synthetic Construct
GRGEAETRECIYYNANWELERTNQSGLERCEGEQDKRLHCYASWRNSSGTIEIVKQGCWLDDETCYDRTDCVEKKDSPQVYFCCCEGNMCNEKFSYFPEMEVTQPTSGGGDKTHTCPPCPAPELLGGPSVFLFPPKPKDTLMISRTPEVTCVVVDVSHEDPEVKFNWYVDGVEVHNAKTKPREEQYNSTYRVVSVLTVLHQDWLNGKEYKCKVSNKALPAPIEKTISKAKGQPREPQVYTLPPSRDELTKNQVSLTCLVKGFYPSDIAVEWESNGQPENNYKTTPPVLDSDGSFFLYSKLTVDKSRWQQGNVFSCSVMHEALHNHYTQKSLSLSPGK

SEQ ID NO: 325 - protein, 339 aa, synthetic construct
  REGION 1..339: note = Synthetic Construct
GAILGRAETRECIYYNANWELERTNQSGLERCEGEQDKRLHCYASWRNSSGTIEIVKQGCWLDDFNCYDRTDCVEKKDSPQVYFCCCEGNMCNEKFSYFPEMEVTQPTSGGGDKTHTCPPCPAPELLGGPSVFLFPPKPKDTLMISRTPEVTCVVVDVSHEDPEVKFNWYVDGVEVHNAKTKPREEQYNSTYRVVSVLTVLHQDWLNGKEYKCKVSNKALPAPIEKTISKAKGQPREPQVYTLPPSRDELTKNQVSLTCLVKGFYPSDIAVEWESNGQPENNYKTTPPVLDSDGSFFLYSKLTVDKSRWQQGNVFSCSVMHEALHNHYTQKSLSLSPGK

SEQ ID NO: 326 - protein, 339 aa, synthetic construct
  REGION 1..339: note = Synthetic Construct
GAILGRSETQECIYYNANWELERTNQSGLERCEGEQDKRLHCYASWRNSSGTIEIVKQGCWLDDFNCYDRTDCVEKKDSPQVYFCCCEGNMCNEKFSYFPEMEVTQPTSGGGDKTHTCPPCPAPELLGGPSVFLFPPKPKDTLMISRTPEVTCVVVDVSHEDPEVKFNWYVDGVEVHNAKTKPREEQYNSTYRVVSVLTVLHQDWLNGKEYKCKVSNKALPAPIEKTISKAKGQPREPQVYTLPPSRDELTKNQVSLTCLVKGFYPSDIAVEWESNGQPENNYKTTPPVLDSDGSFFLYSKLTVDKSRWQQGNVFSCSVMHEALHNHYTQKSLSLSPGK

SEQ ID NO: 327 - protein, 337 aa, synthetic construct
  REGION 1..337: note = Synthetic Construct
GRGEAETRECIYYNANWELERTNQSGLERCEGEQDKRLHCYASWRNSSGTIELVKKGCWLDDFNCYDRQECVATKDSPEVYFCCCEGNMCNEKFSYFPEMEVTQPTSGGGDKTHTCPPCPAPELLGGPSVFLFPPKPKDTLMISRTPEVTCVVVDVSHEDPEVKFNWYVDGVEVHNAKTKPREEQYNSTYRVVSVLTVLHQDWLNGKEYKCKVSNKALPAPIEKTISKAKGQPREPQVYTLPPSRDELTKNQVSLTCLVKGFYPSDIAVEWESNGQPENNYKTTPPVLDSDGSFFLYSKLTVDKSRWQQGNVFSCSVMHEALHNHYTQKSLSLSPGK

SEQ ID NO: 328 - protein, 337 aa, synthetic construct
  REGION 1..337: note = Synthetic Construct
GRGEAETRECIYYNANWELERTNQSGLERCEGEQDKRLHCYASWRNSSGTIELVKKGCWLDDFNCYDRQECVATKENPQVYFCCCEGNMCNEKFSYFPEMEVTQPTSGGGDKTHTCPPCPAPELLGGPSVFLFPPKPKDTLMISRTPEVTCVVVDVSHEDPEVKFNWYVDGVEVHNAKTKPREEQYNSTYRVVSVLTVLHQDWLNGKEYKCKVSNKALPAPIEKTISKAKGQPREPQVYTLPPSRDELTKNQVSLTCLVKGFYPSDIAVEWESNGQPENNYKTTPPVLDSDGSFFLYSKLTVDKSRWQQGNVFSCSVMHEALHNHYTQKSLSLSPGK

SEQ ID NO: 329 - protein, 336 aa, synthetic construct
  REGION 1..336: note = Synthetic Construct
RGEAETRECIYYNANWELERTNQSGLERCEGEQDKRRHCFATWKNISGSIEIVKQGCWLDDFNCYDRTDCVEKKDSPQVYFCCCEGNMCNEKFSYFPEMEVTQPTSGGGDKTHTCPPCPAPELLGGPSVFLFPPKPKDTLMISRTPEVTCVVVDVSHEDPEVKFNWYVDGVEVHNAKTKPREEQYNSTYRVVSVLTVLHQDWLNGKEYKCKVSNKALPAPIEKTISKAKGQPREPQVYTLPPSRDELTKNQVSLTCLVKGFYPSDIAVEWESNGQPENNYKTTPPVLDSDGSFFLYSKLTVDKSRWQQGNVFSCSVMHEALHNHYTQKSLSLSPGK

SEQ ID NO: 330 - protein, 336 aa, synthetic construct
  REGION 1..336: note = Synthetic Construct
RGEAETRECIYYNANWELERTNQSGLERCEGEQDKRLHCYASWRNSSGTIEIVKQGCWLDDETCYDRTDCVEKKDSPQVYFCCCEGNMCNEKFSYFPEMEVTQPTSGGGDKTHTCPPCPAPELLGGPSVFLFPPKPKDTLMISRTPEVTCVVVDVSHEDPEVKFNWYVDGVEVHNAKTKPREEQYNSTYRVVSVLTVLHQDWLNGKEYKCKVSNKALPAPIEKTISKAKGQPREPQVYTLPPSRDELTKNQVSLTCLVKGFYPSDIAVEWESNGQPENNYKTTPPVLDSDGSFFLYSKLTVDKSRWQQGNVFSCSVMHEALHNHYTQKSLSLSPGK

SEQ ID NO: 331 - protein, 337 aa, synthetic construct
  REGION 1..337: note = Synthetic Construct
ILGRAETRECIYYNANWELERTNQSGLERCEGEQDKRLHCYASWRNSSGTIEIVKQGCWLDDFNCYDRTDCVEKKDSPQVYFCCCEGNMCNEKFSYFPEMEVTQPTSGGGDKTHTCPPCPAPELLGGPSVFLFPPKPKDTLMISRTPEVTCVVVDVSHEDPEVKFNWYVDGVEVHNAKTKPREEQYNSTYRVVSVLTVLHQDWLNGKEYKCKVSNKALPAPIEKTISKAKGQPREPQVYTLPPSRDELTKNQVSLTCLVKGFYPSDIAVEWESNGQPENNYKTTPPVLDSDGSFFLYSKLTVDKSRWQQGNVFSCSVMHEALHNHYTQKSLSLSPGK

SEQ ID NO: 332 - protein, 337 aa, synthetic construct
  REGION 1..337: note = Synthetic Construct
ILGRSETQECIYYNANWELERTNQSGLERCEGEQDKRLHCYASWRNSSGTIEIVKQGCWLDDFNCYDRTDCVEKKDSPQVYFCCCEGNMCNEKFSYFPEMEVTQPTSGGGDKTHTCPPCPAPELLGGPSVFLFPPKPKDTLMISRTPEVTCVVVDVSHEDPEVKFNWYVDGVEVHNAKTKPREEQYNSTYRVVSVLTVLHQDWLNGKEYKCKVSNKALPAPIEKTISKAKGQPREPQVYTLPPSRDELTKNQVSLTCLVKGFYPSDIAVEWESNGQPENNYKTTPPVLDSDGSFFLYSKLTVDKSRWQQGNVFSCSVMHEALHNHYTQKSLSLSPGK

SEQ ID NO: 333 - protein, 336 aa, synthetic construct
  REGION 1..336: note = Synthetic Construct
RGEAETRECIYYNANWELERTNQSGLERCEGEQDKRLHCYASWRNSSGTIELVKKGCWLDDFNCYDRQECVATKDSPEVYFCCCEGNMCNEKFSYFPEMEVTQPTSGGGDKTHTCPPCPAPELLGGPSVFLFPPKPKDTLMISRTPEVTCVVVDVSHEDPEVKFNWYVDGVEVHNAKTKPREEQYNSTYRVVSVLTVLHQDWLNGKEYKCKVSNKALPAPIEKTISKAKGQPREPQVYTLPPSRDELTKNQVSLTCLVKGFYPSDIAVEWESNGQPENNYKTTPPVLDSDGSFFLYSKLTVDKSRWQQGNVFSCSVMHEALHNHYTQKSLSLSPGK

SEQ ID NO: 334 - protein, 336 aa, synthetic construct
  REGION 1..336: note = Synthetic Construct
RGEAETRECIYYNANWELERTNQSGLERCEGEQDKRLHCYASWRNSSGTIELVKKGCWLDDFNCYDRQECVATKENPQVYFCCCEGNMCNEKFSYFPEMEVTQPTSGGGDKTHTCPPCPAPELLGGPSVFLFPPKPKDTLMISRTPEVTCVVVDVSHEDPEVKFNWYVDGVEVHNAKTKPREEQYNSTYRVVSVLTVLHQDWLNGKEYKCKVSNKALPAPIEKTISKAKGQPREPQVYTLPPSRDELTKNQVSLTCLVKGFYPSDIAVEWESNGQPENNYKTTPPVLDSDGSFFLYSKLTVDKSRWQQGNVFSCSVMHEALHNHYTQKSLSLSPGK

SEQ ID NO: 335 - protein, 335 aa, synthetic construct
  REGION 1..335: note = Synthetic Construct
GEAETRECIYYNANWELERTNQSGLERCEGEQDKRRHCFATWKNISGSIEIVKQGCWLDDFNCYDRTDCVEKKDSPQVYFCCCEGNMCNEKFSYFPEMEVTQPTSGGGDKTHTCPPCPAPELLGGPSVFLFPPKPKDTLMISRTPEVTCVVVDVSHEDPEVKFNWYVDGVEVHNAKTKPREEQYNSTYRVVSVLTVLHQDWLNGKEYKCKVSNKALPAPIEKTISKAKGQPREPQVYTLPPSRDELTKNQVSLTCLVKGFYPSDIAVEWESNGQPENNYKTTPPVLDSDGSFFLYSKLTVDKSRWQQGNVFSCSVMHEALHNHYTQKSLSLSPGK

SEQ ID NO: 336 - protein, 335 aa, synthetic construct
  REGION 1..335: note = Synthetic Construct
GEAETRECIYYNANWELERTNQSGLERCEGEQDKRLHCYASWRNSSGTIEIVKQGCWLDDETCYDRTDCVEKKDSPQVYFCCCEGNMCNEKFSYFPEMEVTQPTSGGGDKTHTCPPCPAPELLGGPSVFLFPPKPKDTLMISRTPEVTCVVVDVSHEDPEVKFNWYVDGVEVHNAKTKPREEQYNSTYRVVSVLTVLHQDWLNGKEYKCKVSNKALPAPIEKTISKAKGQPREPQVYTLPPSRDELTKNQVSLTCLVKGFYPSDIAVEWESNGQPENNYKTTPPVLDSDGSFFLYSKLTVDKSRWQQGNVFSCSVMHEALHNHYTQKSLSLSPGK

SEQ ID NO: 337 - protein, 336 aa, synthetic construct
  REGION 1..336: note = Synthetic Construct
LGRAETRECIYYNANWELERTNQSGLERCEGEQDKRLHCYASWRNSSGTIEIVKQGCWLDDFNCYDRTDCVEKKDSPQVYFCCCEGNMCNEKFSYFPEMEVTQPTSGGGDKTHTCPPCPAPELLGGPSVFLFPPKPKDTLMISRTPEVTCVVVDVSHEDPEVKFNWYVDGVEVHNAKTKPREEQYNSTYRVVSVLTVLHQDWLNGKEYKCKVSNKALPAPIEKTISKAKGQPREPQVYTLPPSRDELTKNQVSLTCLVKGFYPSDIAVEWESNGQPENNYKTTPPVLDSDGSFFLYSKLTVDKSRWQQGNVFSCSVMHEALHNHYTQKSLSLSPGK

SEQ ID NO: 338 - protein, 336 aa, synthetic construct
  REGION 1..336: note = Synthetic Construct
LGRSETQECIYYNANWELERTNQSGLERCEGEQDKRLHCYASWRNSSGTIEIVKQGCWLDDFNCYDRTDCVEKKDSPQVYFCCCEGNMCNEKFSYFPEMEVTQPTSGGGDKTHTCPPCPAPELLGGPSVFLFPPKPKDTLMISRTPEVTCVVVDVSHEDPEVKFNWYVDGVEVHNAKTKPREEQYNSTYRVVSVLTVLHQDWLNGKEYKCKVSNKALPAPIEKTISKAKGQPREPQVYTLPPSRDELTKNQVSLTCLVKGFYPSDIAVEWESNGQPENNYKTTPPVLDSDGSFFLYSKLTVDKSRWQQGNVFSCSVMHEALHNHYTQKSLSLSPGK

SEQ ID NO: 339 - protein, 335 aa, synthetic construct
  REGION 1..335: note = Synthetic Construct
GEAETRECIYYNANWELERTNQSGLERCEGEQDKRLHCYASWRNSSGTIELVKKGCWLDDFNCYDRQECVATKDSPEVYFCCCEGNMCNEKFSYFPEMEVTQPTSGGGDKTHTCPPCPAPELLGGPSVFLFPPKPKDTLMISRTPEVTCVVVDVSHEDPEVKFNWYVDGVEVHNAKTKPREEQYNSTYRVVSVLTVLHQDWLNGKEYKCKVSNKALPAPIEKTISKAKGQPREPQVYTLPPSRDELTKNQVSLTCLVKGFYPSDIAVEWESNGQPENNYKTTPPVLDSDGSFFLYSKLTVDKSRWQQGNVFSCSVMHEALHNHYTQKSLSLSPGK

SEQ ID NO: 340 - protein, 335 aa, synthetic construct
  REGION 1..335: note = Synthetic Construct
GEAETRECIYYNANWELERTNQSGLERCEGEQDKRLHCYASWRNSSGTIELVKKGCWLDDFNCYDRQECVATKENPQVYFCCCEGNMCNEKFSYFPEMEVTQPTSGGGDKTHTCPPCPAPELLGGPSVFLFPPKPKDTLMISRTPEVTCVVVDVSHEDPEVKFNWYVDGVEVHNAKTKPREEQYNSTYRVVSVLTVLHQDWLNGKEYKCKVSNKALPAPIEKTISKAKGQPREPQVYTLPPSRDELTKNQVSLTCLVKGFYPSDIAVEWESNGQPENNYKTTPPVLDSDGSFFLYSKLTVDKSRWQQGNVFSCSVMHEALHNHYTQKSLSLSPGK

SEQ ID NO: 341 - protein, 334 aa, synthetic construct
  REGION 1..334: note = Synthetic Construct
EAETRECIYYNANWELERTNQSGLERCEGEQDKRRHCFATWKNISGSIEIVKQGCWLDDFNCYDRTDCVEKKDSPQVYFCCCEGNMCNEKFSYFPEMEVTQPTSGGGDKTHTCPPCPAPELLGGPSVFLFPPKPKDTLMISRTPEVTCVVVDVSHEDPEVKFNWYVDGVEVHNAKTKPREEQYNSTYRVVSVLTVLHQDWLNGKEYKCKVSNKALPAPIEKTISKAKGQPREPQVYTLPPSRDELTKNQVSLTCLVKGFYPSDIAVEWESNGQPENNYKTTPPVLDSDGSFFLYSKLTVDKSRWQQGNVFSCSVMHEALHNHYTQKSLSLSPGK

SEQ ID NO: 342 - protein, 334 aa, synthetic construct
  REGION 1..334: note = Synthetic Construct
EAETRECIYYNANWELERTNQSGLERCEGEQDKRLHCYASWRNSSGTIEIVKQGCWLDDETCYDRTDCVEKKDSPQVYFCCCEGNMCNEKFSYFPEMEVTQPTSGGGDKTHTCPPCPAPELLGGPSVFLFPPKPKDTLMISRTPEVTCVVVDVSHEDPEVKFNWYVDGVEVHNAKTKPREEQYNSTYRVVSVLTVLHQDWLNGKEYKCKVSNKALPAPIEKTISKAKGQPREPQVYTLPPSRDELTKNQVSLTCLVKGFYPSDIAVEWESNGQPENNYKTTPPVLDSDGSFFLYSKLTVDKSRWQQGNVFSCSVMHEALHNHYTQKSLSLSPGK

SEQ ID NO: 343 - protein, 335 aa, synthetic construct
  REGION 1..335: note = Synthetic Construct
GRAETRECIYYNANWELERTNQSGLERCEGEQDKRLHCYASWRNSSGTIEIVKQGCWLDDFNCYDRTDCVEKKDSPQVYFCCCEGNMCNEKFSYFPEMEVTQPTSGGGDKTHTCPPCPAPELLGGPSVFLFPPKPKDTLMISRTPEVTCVVVDVSHEDPEVKFNWYVDGVEVHNAKTKPREEQYNSTYRVVSVLTVLHQDWLNGKEYKCKVSNKALPAPIEKTISKAKGQPREPQVYTLPPSRDELTKNQVSLTCLVKGFYPSDIAVEWESNGQPENNYKTTPPVLDSDGSFFLYSKLTVDKSRWQQGNVFSCSVMHEALHNHYTQKSLSLSPGK

SEQ ID NO: 344 - protein, 335 aa, synthetic construct
  REGION 1..335: note = Synthetic Construct
GRSETQECIYYNANWELERTNQSGLERCEGEQDKRLHCYASWRNSSGTIEIVKQGCWLDDFNCYDRTDCVEKKDSPQVYFCCCEGNMCNEKFSYFPEMEVTQPTSGGGDKTHTCPPCPAPELLGGPSVFLFPPKPKDTLMISRTPEVTCVVVDVSHEDPEVKFNWYVDGVEVHNAKTKPREEQYNSTYRVVSVLTVLHQDWLNGKEYKCKVSNKALPAPIEKTISKAKGQPREPQVYTLPPSRDELTKNQVSLTCLVKGFYPSDIAVEWESNGQPENNYKTTPPVLDSDGSFFLYSKLTVDKSRWQQGNVFSCSVMHEALHNHYTQKSLSLSPGK

SEQ ID NO: 345 - protein, 334 aa, synthetic construct
  REGION 1..334: note = Synthetic Construct
EAETRECIYYNANWELERTNQSGLERCEGEQDKRLHCYASWRNSSGTIELVKKGCWLDDFNCYDRQECVATKDSPEVYFCCCEGNMCNEKFSYFPEMEVTQPTSGGGDKTHTCPPCPAPELLGGPSVFLFPPKPKDTLMISRTPEVTCVVVDVSHEDPEVKFNWYVDGVEVHNAKTKPREEQYNSTYRVVSVLTVLHQDWLNGKEYKCKVSNKALPAPIEKTISKAKGQPREPQVYTLPPSRDELTKNQVSLTCLVKGFYPSDIAVEWESNGQPENNYKTTPPVLDSDGSFFLYSKLTVDKSRWQQGNVFSCSVMHEALHNHYTQKSLSLSPGK

SEQ ID NO: 346 - protein, 334 aa, synthetic construct
  REGION 1..334: note = Synthetic Construct
EAETRECIYYNANWELERTNQSGLERCEGEQDKRLHCYASWRNSSGTIELVKKGCWLDDFNCYDRQECVATKENPQVYFCCCEGNMCNEKFSYFPEMEVTQPTSGGGDKTHTCPPCPAPELLGGPSVFLFPPKPKDTLMISRTPEVTCVVVDVSHEDPEVKFNWYVDGVEVHNAKTKPREEQYNSTYRVVSVLTVLHQDWLNGKEYKCKVSNKALPAPIEKTISKAKGQPREPQVYTLPPSRDELTKNQVSLTCLVKGFYPSDIAVEWESNGQPENNYKTTPPVLDSDGSFFLYSKLTVDKSRWQQGNVFSCSVMHEALHNHYTQKSLSLSPGK

SEQ ID NO: 347 - protein, 333 aa, synthetic construct
  REGION 1..333: note = Synthetic Construct
AETRECIYYNANWELERTNQSGLERCEGEQDKRRHCFATWKNISGSIEIVKQGCWLDDFNCYDRTDCVEKKDSPQVYFCCCEGNMCNEKFSYFPEMEVTQPTSGGGDKTHTCPPCPAPELLGGPSVFLFPPKPKDTLMISRTPEVTCVVVDVSHEDPEVKFNWYVDGVEVHNAKTKPREEQYNSTYRVVSVLTVLHQDWLNGKEYKCKVSNKALPAPIEKTISKAKGQPREPQVYTLPPSRDELTKNQVSLTCLVKGFYPSDIAVEWESNGQPENNYKTTPPVLDSDGSFFLYSKLTVDKSRWQQGNVFSCSVMHEALHNHYTQKSLSLSPGK

SEQ ID NO: 348 - protein, 333 aa, synthetic construct
  REGION 1..333: note = Synthetic Construct
AETRECIYYNANWELERTNQSGLERCEGEQDKRLHCYASWRNSSGTIEIVKQGCWLDDETCYDRTDCVEKKDSPQVYFCCCEGNMCNEKFSYFPEMEVTQPTSGGGDKTHTCPPCPAPELLGGPSVFLFPPKPKDTLMISRTPEVTCVVVDVSHEDPEVKFNWYVDGVEVHNAKTKPREEQYNSTYRVVSVLTVLHQDWLNGKEYKCKVSNKALPAPIEKTISKAKGQPREPQVYTLPPSRDELTKNQVSLTCLVKGFYPSDIAVEWESNGQPENNYKTTPPVLDSDGSFFLYSKLTVDKSRWQQGNVFSCSVMHEALHNHYTQKSLSLSPGK

SEQ ID NO: 349 - protein, 334 aa, synthetic construct
  REGION 1..334: note = Synthetic Construct
RAETRECIYYNANWELERTNQSGLERCEGEQDKRLHCYASWRNSSGTIEIVKQGCWLDDFNCYDRTDCVEKKDSPQVYFCCCEGNMCNEKFSYFPEMEVTQPTSGGGDKTHTCPPCPAPELLGGPSVFLFPPKPKDTLMISRTPEVTCVVVDVSHEDPEVKFNWYVDGVEVHNAKTKPREEQYNSTYRVVSVLTVLHQDWLNGKEYKCKVSNKALPAPIEKTISKAKGQPREPQVYTLPPSRDELTKNQVSLTCLVKGFYPSDIAVEWESNGQPENNYKTTPPVLDSDGSFFLYSKLTVDKSRWQQGNVFSCSVMHEALHNHYTQKSLSLSPGK

SEQ ID NO: 350 - protein, 334 aa, synthetic construct
  REGION 1..334: note = Synthetic Construct
RSETQECIYYNANWELERTNQSGLERCEGEQDKRLHCYASWRNSSGTIEIVKQGCWLDDFNCYDRTDCVEKKDSPQVYFCCCEGNMCNEKFSYFPEMEVTQPTSGGGDKTHTCPPCPAPELLGGPSVFLFPPKPKDTLMISRTPEVTCVVVDVSHEDPEVKFNWYVDGVEVHNAKTKPREEQYNSTYRVVSVLTVLHQDWLNGKEYKCKVSNKALPAPIEKTISKAKGQPREPQVYTLPPSRDELTKNQVSLTCLVKGFYPSDIAVEWESNGQPENNYKTTPPVLDSDGSFFLYSKLTVDKSRWQQGNVFSCSVMHEALHNHYTQKSLSLSPGK

SEQ ID NO: 351 - protein, 333 aa, synthetic construct
  REGION 1..333: note = Synthetic Construct
AETRECIYYNANWELERTNQSGLERCEGEQDKRLHCYASWRNSSGTIELVKKGCWLDDFNCYDRQECVATKDSPEVYFCCCEGNMCNEKFSYFPEMEVTQPTSGGGDKTHTCPPCPAPELLGGPSVFLFPPKPKDTLMISRTPEVTCVVVDVSHEDPEVKFNWYVDGVEVHNAKTKPREEQYNSTYRVVSVLTVLHQDWLNGKEYKCKVSNKALPAPIEKTISKAKGQPREPQVYTLPPSRDELTKNQVSLTCLVKGFYPSDIAVEWESNGQPENNYKTTPPVLDSDGSFFLYSKLTVDKSRWQQGNVFSCSVMHEALHNHYTQKSLSLSPGK

SEQ ID NO: 352 - protein, 333 aa, synthetic construct
  REGION 1..333: note = Synthetic Construct
AETRECIYYNANWELERTNQSGLERCEGEQDKRLHCYASWRNSSGTIELVKKGCWLDDFNCYDRQECVATKENPQVYFCCCEGNMCNEKFSYFPEMEVTQPTSGGGDKTHTCPPCPAPELLGGPSVFLFPPKPKDTLMISRTPEVTCVVVDVSHEDPEVKFNWYVDGVEVHNAKTKPREEQYNSTYRVVSVLTVLHQDWLNGKEYKCKVSNKALPAPIEKTISKAKGQPREPQVYTLPPSRDELTKNQVSLTCLVKGFYPSDIAVEWESNGQPENNYKTTPPVLDSDGSFFLYSKLTVDKSRWQQGNVFSCSVMHEALHNHYTQKSLSLSPGK

SEQ ID NO: 353 - protein, 332 aa, synthetic construct
  REGION 1..332: note = Synthetic Construct
ETRECIYYNANWELERTNQSGLERCEGEQDKRRHCFATWKNISGSIEIVKQGCWLDDFNCYDRTDCVEKKDSPQVYFCCCEGNMCNEKFSYFPEMEVTQPTSGGGDKTHTCPPCPAPELLGGPSVFLFPPKPKDTLMISRTPEVTCVVVDVSHEDPEVKFNWYVDGVEVHNAKTKPREEQYNSTYRVVSVLTVLHQDWLNGKEYKCKVSNKALPAPIEKTISKAKGQPREPQVYTLPPSRDELTKNQVSLTCLVKGFYPSDIAVEWESNGQPENNYKTTPPVLDSDGSFFLYSKLTVDKSRWQQGNVFSCSVMHEALHNHYTQKSLSLSPGK

SEQ ID NO: 354 - protein, 332 aa, synthetic construct
  REGION 1..332: note = Synthetic Construct
ETRECIYYNANWELERTNQSGLERCEGEQDKRLHCYASWRNSSGTIEIVKQGCWLDDETCYDRTDCVEKKDSPQVYFCCCEGNMCNEKFSYFPEMEVTQPTSGGGDKTHTCPPCPAPELLGGPSVFLFPPKPKDTLMISRTPEVTCVVVDVSHEDPEVKFNWYVDGVEVHNAKTKPREEQYNSTYRVVSVLTVLHQDWLNGKEYKCKVSNKALPAPIEKTISKAKGQPREPQVYTLPPSRDELTKNQVSLTCLVKGFYPSDIAVEWESNGQPENNYKTTPPVLDSDGSFFLYSKLTVDKSRWQQGNVFSCSVMHEALHNHYTQKSLSLSPGK

SEQ ID NO: 355 - protein, 333 aa, synthetic construct; identical to SEQ ID NO: 309
  REGION 1..333: note = Synthetic Construct

SEQ ID NO: 356 - protein, 333 aa, synthetic construct
  REGION 1..333: note = Synthetic Construct
SETQECIYYNANWELERTNQSGLERCEGEQDKRLHCYASWRNSSGTIEIVKQGCWLDDFNCYDRTDCVEKKDSPQVYFCCCEGNMCNEKFSYFPEMEVTQPTSGGGDKTHTCPPCPAPELLGGPSVFLFPPKPKDTLMISRTPEVTCVVVDVSHEDPEVKFNWYVDGVEVHNAKTKPREEQYNSTYRVVSVLTVLHQDWLNGKEYKCKVSNKALPAPIEKTISKAKGQPREPQVYTLPPSRDELTKNQVSLTCLVKGFYPSDIAVEWESNGQPENNYKTTPPVLDSDGSFFLYSKLTVDKSRWQQGNVFSCSVMHEALHNHYTQKSLSLSPGK

SEQ ID NO: 357 - protein, 332 aa, synthetic construct
  REGION 1..332: note = Synthetic Construct
ETRECIYYNANWELERTNQSGLERCEGEQDKRLHCYASWRNSSGTIELVKKGCWLDDFNCYDRQECVATKDSPEVYFCCCEGNMCNEKFSYFPEMEVTQPTSGGGDKTHTCPPCPAPELLGGPSVFLFPPKPKDTLMISRTPEVTCVVVDVSHEDPEVKFNWYVDGVEVHNAKTKPREEQYNSTYRVVSVLTVLHQDWLNGKEYKCKVSNKALPAPIEKTISKAKGQPREPQVYTLPPSRDELTKNQVSLTCLVKGFYPSDIAVEWESNGQPENNYKTTPPVLDSDGSFFLYSKLTVDKSRWQQGNVFSCSVMHEALHNHYTQKSLSLSPGK

SEQ ID NO: 358 - protein, 332 aa, synthetic construct
  REGION 1..332: note = Synthetic Construct
ETRECIYYNANWELERTNQSGLERCEGEQDKRLHCYASWRNSSGTIELVKKGCWLDDFNCYDRQECVATKENPQVYFCCCEGNMCNEKFSYFPEMEVTQPTSGGGDKTHTCPPCPAPELLGGPSVFLFPPKPKDTLMISRTPEVTCVVVDVSHEDPEVKFNWYVDGVEVHNAKTKPREEQYNSTYRVVSVLTVLHQDWLNGKEYKCKVSNKALPAPIEKTISKAKGQPREPQVYTLPPSRDELTKNQVSLTCLVKGFYPSDIAVEWESNGQPENNYKTTPPVLDSDGSFFLYSKLTVDKSRWQQGNVFSCSVMHEALHNHYTQKSLSLSPGK

SEQ ID NO: 359 - protein, 331 aa, synthetic construct
  REGION 1..331: note = Synthetic Construct
TRECIYYNANWELERTNQSGLERCEGEQDKRRHCFATWKNISGSIEIVKQGCWLDDFNCYDRTDCVEKKDSPQVYFCCCEGNMCNEKFSYFPEMEVTQPTSGGGDKTHTCPPCPAPELLGGPSVFLFPPKPKDTLMISRTPEVTCVVVDVSHEDPEVKFNWYVDGVEVHNAKTKPREEQYNSTYRVVSVLTVLHQDWLNGKEYKCKVSNKALPAPIEKTISKAKGQPREPQVYTLPPSRDELTKNQVSLTCLVKGFYPSDIAVEWESNGQPENNYKTTPPVLDSDGSFFLYSKLTVDKSRWQQGNVFSCSVMHEALHNHYTQKSLSLSPGK

SEQ ID NO: 360 - protein, 331 aa, synthetic construct
  REGION 1..331: note = Synthetic Construct
TRECIYYNANWELERTNQSGLERCEGEQDKRLHCYASWRNSSGTIEIVKQGCWLDDETCYDRTDCVEKKDSPQVYFCCCEGNMCNEKFSYFPEMEVTQPTSGGGDKTHTCPPCPAPELLGGPSVFLFPPKPKDTLMISRTPEVTCVVVDVSHEDPEVKFNWYVDGVEVHNAKTKPREEQYNSTYRVVSVLTVLHQDWLNGKEYKCKVSNKALPAPIEKTISKAKGQPREPQVYTLPPSRDELTKNQVSLTCLVKGFYPSDIAVEWESNGQPENNYKTTPPVLDSDGSFFLYSKLTVDKSRWQQGNVFSCSVMHEALHNHYTQKSLSLSPGK

SEQ ID NO: 361 - protein, 330 aa, synthetic construct
  REGION 1..330: note = Synthetic Construct
QECIYYNANWELERTNQSGLERCEGEQDKRLHCYASWRNSSGTIEIVKQGCWLDDFNCYDRTDCVEKKDSPQVYFCCCEGNMCNEKFSYFPEMEVTQPTSGGGDKTHTCPPCPAPELLGGPSVFLFPPKPKDTLMISRTPEVTCVVVDVSHEDPEVKFNWYVDGVEVHNAKTKPREEQYNSTYRVVSVLTVLHQDWLNGKEYKCKVSNKALPAPIEKTISKAKGQPREPQVYTLPPSRDELTKNQVSLTCLVKGFYPSDIAVEWESNGQPENNYKTTPPVLDSDGSFFLYSKLTVDKSRWQQGNVFSCSVMHEALHNHYTQKSLSLSPGK

SEQ ID NO: 362 - protein, 332 aa, synthetic construct; identical to SEQ ID NO: 313
  REGION 1..332: note = Synthetic Construct

SEQ ID NO: 363 - protein, 332 aa, synthetic construct
  REGION 1..332: note = Synthetic Construct
ETQECIYYNANWELERTNQSGLERCEGEQDKRLHCYASWRNSSGTIEIVKQGCWLDDFNCYDRTDCVEKKDSPQVYFCCCEGNMCNEKFSYFPEMEVTQPTSGGGDKTHTCPPCPAPELLGGPSVFLFPPKPKDTLMISRTPEVTCVVVDVSHEDPEVKFNWYVDGVEVHNAKTKPREEQYNSTYRVVSVLTVLHQDWLNGKEYKCKVSNKALPAPIEKTISKAKGQPREPQVYTLPPSRDELTKNQVSLTCLVKGFYPSDIAVEWESNGQPENNYKTTPPVLDSDGSFFLYSKLTVDKSRWQQGNVFSCSVMHEALHNHYTQKSLSLSPGK

SEQ ID NO: 364 - protein, 331 aa, synthetic construct
  REGION 1..331: note = Synthetic Construct
TRECIYYNANWELERTNQSGLERCEGEQDKRLHCYASWRNSSGTIELVKKGCWLDDFNCYDRQECVATKDSPEVYFCCCEGNMCNEKFSYFPEMEVTQPTSGGGDKTHTCPPCPAPELLGGPSVFLFPPKPKDTLMISRTPEVTCVVVDVSHEDPEVKFNWYVDGVEVHNAKTKPREEQYNSTYRVVSVLTVLHQDWLNGKEYKCKVSNKALPAPIEKTISKAKGQPREPQVYTLPPSRDELTKNQVSLTCLVKGFYPSDIAVEWESNGQPENNYKTTPPVLDSDGSFFLYSKLTVDKSRWQQGNVFSCSVMHEALHNHYTQKSLSLSPGK

SEQ ID NO: 365 - protein, 331 aa, synthetic construct
  REGION 1..331: note = Synthetic Construct
TRECIYYNANWELERTNQSGLERCEGEQDKRLHCYASWRNSSGTIELVKKGCWLDDFNCYDRQECVATKENPQVYFCCCEGNMCNEKFSYFPEMEVTQPTSGGGDKTHTCPPCPAPELLGGPSVFLFPPKPKDTLMISRTPEVTCVVVDVSHEDPEVKFNWYVDGVEVHNAKTKPREEQYNSTYRVVSVLTVLHQDWLNGKEYKCKVSNKALPAPIEKTISKAKGQPREPQVYTLPPSRDELTKNQVSLTCLVKGFYPSDIAVEWESNGQPENNYKTTPPVLDSDGSFFLYSKLTVDKSRWQQGNVFSCSVMHEALHNHYTQKSLSLSPGK

SEQ ID NO: 366 - protein, 330 aa, synthetic construct
  REGION 1..330: note = Synthetic Construct
RECIYYNANWELERTNQSGLERCEGEQDKRRHCFATWKNISGSIEIVKQGCWLDDFNCYDRTDCVEKKDSPQVYFCCCEGNMCNEKFSYFPEMEVTQPTSGGGDKTHTCPPCPAPELLGGPSVFLFPPKPKDTLMISRTPEVTCVVVDVSHEDPEVKFNWYVDGVEVHNAKTKPREEQYNSTYRVVSVLTVLHQDWLNGKEYKCKVSNKALPAPIEKTISKAKGQPREPQVYTLPPSRDELTKNQVSLTCLVKGFYPSDIAVEWESNGQPENNYKTTPPVLDSDGSFFLYSKLTVDKSRWQQGNVFSCSVMHEALHNHYTQKSLSLSPGK

SEQ ID NO: 367 - protein, 330 aa, synthetic construct
  REGION 1..330: note = Synthetic Construct
RECIYYNANWELERTNQSGLERCEGEQDKRLHCYASWRNSSGTIEIVKQGCWLDDETCYDRTDCVEKKDSPQVYFCCCEGNMCNEKFSYFPEMEVTQPTSGGGDKTHTCPPCPAPELLGGPSVFLFPPKPKDTLMISRTPEVTCVVVDVSHEDPEVKFNWYVDGVEVHNAKTKPREEQYNSTYRVVSVLTVLHQDWLNGKEYKCKVSNKALPAPIEKTISKAKGQPREPQVYTLPPSRDELTKNQVSLTCLVKGFYPSDIAVEWESNGQPENNYKTTPPVLDSDGSFFLYSKLTVDKSRWQQGNVFSCSVMHEALHNHYTQKSLSLSPGK

SEQ ID NO: 368 - protein, 331 aa, synthetic construct; identical to SEQ ID NO: 317
  REGION 1..331: note = Synthetic Construct

SEQ ID NO: 369 - protein, 331 aa, synthetic construct
  REGION 1..331: note = Synthetic Construct
TQECIYYNANWELERTNQSGLERCEGEQDKRLHCYASWRNSSGTIEIVKQGCWLDDFNCYDRTDCVEKKDSPQVYFCCCEGNMCNEKFSYFPEMEVTQPTSGGGDKTHTCPPCPAPELLGGPSVFLFPPKPKDTLMISRTPEVTCVVVDVSHEDPEVKFNWYVDGVEVHNAKTKPREEQYNSTYRVVSVLTVLHQDWLNGKEYKCKVSNKALPAPIEKTISKAKGQPREPQVYTLPPSRDELTKNQVSLTCLVKGFYPSDIAVEWESNGQPENNYKTTPPVLDSDGSFFLYSKLTVDKSRWQQGNVFSCSVMHEALHNHYTQKSLSLSPGK

SEQ ID NO: 370 - protein, 330 aa, synthetic construct
  REGION 1..330: note = Synthetic Construct
RECIYYNANWELERTNQSGLERCEGEQDKRLHCYASWRNSSGTIELVKKGCWLDDFNCYDRQECVATKDSPEVYFCCCEGNMCNEKFSYFPEMEVTQPTSGGGDKTHTCPPCPAPELLGGPSVFLFPPKPKDTLMISRTPEVTCVVVDVSHEDPEVKFNWYVDGVEVHNAKTKPREEQYNSTYRVVSVLTVLHQDWLNGKEYKCKVSNKALPAPIEKTISKAKGQPREPQVYTLPPSRDELTKNQVSLTCLVKGFYPSDIAVEWESNGQPENNYKTTPPVLDSDGSFFLYSKLTVDKSRWQQGNVFSCSVMHEALHNHYTQKSLSLSPGK

SEQ ID NO: 371 - protein, 330 aa, synthetic construct
  REGION 1..330: note = Synthetic Construct
RECIYYNANWELERTNQSGLERCEGEQDKRLHCYASWRNSSGTIELVKKGCWLDDFNCYDRQECVATKENPQVYFCCCEGNMCNEKFSYFPEMEVTQPTSGGGDKTHTCPPCPAPELLGGPSVFLFPPKPKDTLMISRTPEVTCVVVDVSHEDPEVKFNWYVDGVEVHNAKTKPREEQYNSTYRVVSVLTVLHQDWLNGKEYKCKVSNKALPAPIEKTISKAKGQPREPQVYTLPPSRDELTKNQVSLTCLVKGFYPSDIAVEWESNGQPENNYKTTPPVLDSDGSFFLYSKLTVDKSRWQQGNVFSCSVMHEALHNHYTQKSLSLSPGK

SEQ ID NO: 372 - protein, 330 aa, synthetic construct; identical to SEQ ID NO: 321
  REGION 1..330: note = Synthetic Construct

SEQ ID NO: 373 - protein, 337 aa, synthetic construct
  REGION 1..337: note = Synthetic Construct
GRGEAETRECIYYNANWELERTNQSGLERCEGEQRKRLHCYASWRNSSGTIEIVKQGCWLDDFNCYDRTDCVEKKDSPQVYFCCCEGNMCNEKFSYFPEMEVTQPTSGGGDKTHTCPPCPAPELLGGPSVFLFPPKPKDTLMISRTPEVTCVVVDVSHEDPEVKFNWYVDGVEVHNAKTKPREEQYNSTYRVVSVLTVLHQDWLNGKEYKCKVSNKALPAPIEKTISKAKGQPREPQVYTLPPSRDELTKNQVSLTCLVKGFYPSDIAVEWESNGQPENNYKTTPPVLDSDGSFFLYSKLTVDKSRWQQGNVFSCSVMHEALHNHYTQKSLSLSPGK

SEQ ID NO: 374 - protein, 4 aa, synthetic construct
  REGION 1..4: note = Synthetic Construct
TEEN

SEQ ID NO: 375 - protein, 4 aa, synthetic construct
  REGION 1..4: note = Synthetic Construct
TKEN

SEQ ID NO: 376 - DNA, 22 bp, synthetic construct
  misc_feature 1..22: note = Synthetic Construct
  source 1..22: mol_type = other DNA
ttcagcggattctggagtgcct

SEQ ID NO: 377 - DNA, 22 bp, synthetic construct
  misc_feature 1..22: note = Synthetic Construct
  source 1..22: mol_type = other DNA
agcaacagcgagatgaggacca

SEQ ID NO: 378 - DNA, 17 bp, synthetic construct
  misc_feature 1..17: note = Synthetic Construct
  source 1..17: mol_type = other DNA
catcgtgggccgcccta

SEQ ID NO: 379 - DNA, 22 bp, synthetic construct
  misc_feature 1..22: note = Synthetic Construct
  source 1..22: mol_type = other DNA
cacccacataggagtccttctg

SEQ ID NO: 380 - protein, 4 aa, synthetic construct
KKDS

SEQ ID NO: 381 - protein, 4 aa, synthetic construct
TKDS

SEQ ID NO: 382 - protein, 10 aa, synthetic construct
  VARIANT 1: note = Any amino acid
  VARIANT 3: note = Any amino acid
  VARIANT 5: note = Any amino acid
  VARIANT 7: note = Any amino acid
  VARIANT 9: note = Any amino acid
  VARIANT 1..10: note = This sequence may encompass 1-5 XP repeating units
XPXPXPXPXP

SEQ ID NO: 383 - protein, 81 aa, Homo sapiens
CLFFNANWEKDRTNQTGVEPCYGDKDKRRHCFATWKNISGSIEIVKQGCWLDDINCYDRTDCVEKKDSPEVYFCCCEGNMC

SEQ ID NO: 384 - protein, 81 aa, Homo sapiens
CIYYNANWELERTNQSGLERCEGEQDKRLHCYASWRNSSGTIELVKKGCWLDDFNCYDRQECVATEENPQVYFCCCEGNFC

SEQ ID NO: 385 - protein, 6 aa, synthetic construct
HHHHHH